European Patent Specification EP 2 838 548 B1, published July 19, 2023. Title: HLA Class II Deficient Cells. Applicant: University of Washington Russell, David W. The sequence listing filed with the application follows.

SEQUENCE LISTING (56 sequences)

SEQ ID NO: 1 - DNA, 987 bp, Homo sapiens
  CDS (61)..(420)
aatataagtggaggcgtcgcgctggcgggcattcctgaagctgacagcattcgggccgagatgtctcgctccgtggccttagctgtgctcgcgctactctctctttctggcctggaggctatccagcgtactccaaagattcaggtttactcacgtcatccagcagagaatggaaagtcaaatttcctgaattgctatgtgtctgggtttcatccatccgacattgaagttgacttactgaagaatggagagagaattgaaaaagtggagcattcagacttgtctttcagcaaggactggtctttctatctcttgtactacactgaattcacccccactgaaaaagatgagtatgcctgccgtgtgaaccatgtgactttgtcacagcccaagatagttaagtgggatcgagacatgtaagcagcatcatggaggtttgaagatgccgcatttggattggatgaattccaaattctgcttgcttgctttttaatattgatatgcttatacacttacactttatgcacaaaatgtagggttataataatgttaacatggacatgatcttctttataattctactttgagtgctgtctccatgtttgatgtatctgagcaggttgctccacaggtagctctaggagggctggcaacttagaggtggggagcagagaattctcttatccaacatcaacatcttggtcagatttgaactcttcaatctcttgcactcaaagcttgttaagatagttaagcgtgcataagttaacttccaatttacatactctgcttagaatttgggggaaaatttagaaatataattgacaggattattggaaatttgttataatgaatgaaacattttgtcatataagattcatatttacttcttatacatttgataaagtaaggcatggttgtggttaatctggtttatttttgttccacaagttaaataaatcataaaacttgatgtgttatctctta

SEQ ID NO: 2 - protein, 119 aa, Homo sapiens
MSRSVALAVLALLSLSGLEAIQRTPKIQVYSRHPAENGKSNFLNCYVSGFHPSDIEVDLLKNGERIEKVEHSDLSFSKDWSFYLLYYTEFTPTEKDEYACRVNHVTLSQPKIVKWDRDM

SEQ ID NO: 3 - DNA, 1611 bp, Homo sapiens
  CDS (85)..(1182)
gagaagccaatcagtgtcgtcgcggtcgctgttctaaagtccgcacgcacccaccgggactcagattctccccagacgccgaggatggccgtcatggcgccccgaaccctcctcctgctactctcgggggccctggccctgacccagacctgggcgggctcccactccatgaggtatttcttcacatccgtgtcccggcccggccgcggggagccccgcttcatcgccgtgggctacgtggacgacacgcagttcgtgcggttcgacagcgacgccgcgagccagaagatggagccgcgggcgccgtggatagagcaggaggggccggagtattgggaccaggagacacggaatatgaaggcccactcacagactgaccgagcgaacctggggaccctgcgcggctactacaaccagagcgaggacggttctcacaccatccagataatgtatggctgcgacgtggggccggacgggcgcttcctccgcgggtaccggcaggacgcctacgacggcaaggattacatcgccctgaacgaggacctgcgctcttggaccgcggcggacatggcagctcagatcaccaagcgcaagtgggaggcggtccatgcggcggagcagcggagagtctacctggagggccggtgcgtggacgggctccgcagatacctggagaacgggaaggagacgctgcagcgcacggacccccccaagacacatatgacccaccaccccatctctgaccatgaggccaccctgaggtgctgggccctgggcttctaccctgcggagatcacactgacctggcagcgggatggggaggaccagacccaggacacggagctcgtggagaccaggcctgcaggggatggaaccttccagaagtgggcggctgtggtggtgccttctggagaggagcagagatacacctgccatgtgcagcatgagggtctgcccaagcccctcaccctgagatgggagctgtcttcccagcccaccatccccatcgtgggcatcattgctggcctggttctccttggagctgtgatcactggagctgtggtcgctgccgtgatgtggaggaggaagagctcagatagaaaaggagggagttacactcaggctgcaagcagtgacagtgcccagggctctgatgtgtctctcacagcttgtaaagtgtgagacagctgccttgtgtgggactgagaggcaagagttgttcctgcccttccctttgtgacttgaagaaccctgactttgtttctgcaaaggcacctgcatgtgtctgtgttcgtgtaggcataatgtgaggaggtggggagagcaccccacccccatgtccaccatgaccctcttcccacgctgacctgtgctccctctccaatcatctttcctgttccagagaggtggggctgaggtgtctccatctctgtctcaacttcatggtgcactgagctgtaacttcttccttccctattaaaattagaacctgagtataaatttactttctcaaattcttgccatgagaggttgatgagttaattaaaggagaagattcctaaaatttgagagacaaaattaatggaacgcatgagaaccttccagagtcca

SEQ ID NO: 4 - protein, 365 aa, Homo sapiens
MAVMAPRTLLLLLSGALALTQTWAGSHSMRYFFTSVSRPGRGEPRFIAVGYVDDTQFVRFDSDAASQKMEPRAPWIEQEGPEYWDQETRNMKAHSQTDRANLGTLRGYYNQSEDGSHTIQIMYGCDVGPDGRFLRGYRQDAYDGKDYIALNEDLRSWTAADMAAQITKRKWEAVHAAEQRRVYLEGRCVDGLRRYLENGKETLQRTDPPKTHMTHHPISDHEATLRCWALGFYPAEITLTWQRDGEDQTQDTELVETRPAGDGTFQKWAAVVVPSGEEQRYTCHVQHEGLPKPLTLRWELSSQPTIPIVGIIAGLVLLGAVITGAVVAAVMWRRKSSDRKGGSYTQAASSDSAQGSDVSLTACKV

SEQ ID NO: 5 - DNA, 1578 bp, Homo sapiens
  CDS (55)..(1143)
agttctaaagtccccacgcacccacccggactcagagtctcctcagacgccgagatgctggtcatggcgccccgaaccgtcctcctgctgctctcggcggccctggccctgaccgagacctgggccggctcccactccatgaggtatttctacacctccgtgtcccggcccggccgcggggagccccgcttcatctcagtgggctacgtggacgacacccagttcgtgaggttcgacagcgacgccgcgagtccgagagaggagccgcgggcgccgtggatagagcaggaggggccggagtattgggaccggaacacacagatctacaaggcccaggcacagactgaccgagagagcctgcggaacctgcgcggctactacaaccagagcgaggccgggtctcacaccctccagagcatgtacggctgcgacgtggggccggacgggcgcctcctccgcgggcatgaccagtacgcctacgacggcaaggattacatcgccctgaacgaggacctgcgctcctggaccgccgcggacacggcggctcagatcacccagcgcaagtgggaggcggcccgtgaggcggagcagcggagagcctacctggagggcgagtgcgtggagtggctccgcagatacctggagaacgggaaggacaagctggagcgcgctgaccccccaaagacacacgtgacccaccaccccatctctgaccatgaggccaccctgaggtgctgggccctgggtttctaccctgcggagatcacactgacctggcagcgggatggcgaggaccaaactcaggacactgagcttgtggagaccagaccagcaggagatagaaccttccagaagtgggcagctgtggtggtgccttctggagaagagcagagatacacatgccatgtacagcatgaggggctgccgaagcccctcaccctgagatgggagccgtcttcccagtccaccgtccccatcgtgggcattgttgctggcctggctgtcctagcagttgtggtcatcggagctgtggtcgctgctgtgatgtgtaggaggaagagttcaggtggaaaaggagggagctactctcaggctgcgtgcagcgacagtgcccagggctctgatgtgtctctcacagcttgaaaagcctgagacagctgtcttgtgagggactgagatgcaggatttcttcacgcctcccctttgtgacttcaagagcctctggcatctctttctgcaaaggcacctgaatgtgtctgcgtccctgttagcataatgtgaggaggtggagagacagcccacccttgtgtccactgtgacccctgttcccatgctgacctgtgtttcctccccagtcatctttcttgttccagagaggtggggctggatgtctccatctctgtctcaactttacgtgcactgagctgcaacttcttacttccctactgaaaataagaatctgaatataaatttgttttctcaaatatttgctatgagaggttgatggattaattaaataagtcaattcctggaatttgagagagcaaataaagacctgagaaccttccagaaaaaaaa

SEQ ID NO: 6 - protein, 362 aa, Homo sapiens
MLVMAPRTVLLLLSAALALTETWAGSHSMRYFYTSVSRPGRGEPRFISVGYVDDTQFVRFDSDAASPREEPRAPWIEQEGPEYWDRNTQIYKAQAQTDRESLRNLRGYYNQSEAGSHTLQSMYGCDVGPDGRLLRGHDQYAYDGKDYIALNEDLRSWTAADTAAQITQRKWEAAREAEQRRAYLEGECVEWLRRYLENGKDKLERADPPKTHVTHHPISDHEATLRCWALGFYPAEITLTWQRDGEDQTQDTELVETRPAGDRTFQKWAAVVVPSGEEQRYTCHVQHEGLPKPLTLRWEPSSQSTVPIVGIVAGLAVLAVVVIGAVVAAVMCRRKSSGGKGGSYSQAACSDSAQGSDVSLTA

SEQ ID NO: 7 - DNA, 1586 bp, Homo sapiens
  CDS (66)..(1166)
tccgcagtcccggttctaaagtccccagtcacccacccggactcacattctccccagaggccgagatgcgggtcatggcgccccgagccctcctcctgctgctctcgggaggcctggccctgaccgagacctgggcctgctcccactccatgaggtatttcgacaccgccgtgtcccggcccggccgcggagagccccgcttcatctcagtgggctacgtggacgacacgcagttcgtgcggttcgacagcgacgccgcgagtccgagaggggagccgcgggcgccgtgggtggagcaggaggggccggagtattgggaccgggagacacagaagtacaagcgccaggcacaggctgaccgagtgagcctgcggaacctgcgcggctactacaaccagagcgaggacgggtctcacaccctccagaggatgtctggctgcgacctggggcccgacgggcgcctcctccgcgggtatgaccagtccgcctacgacggcaaggattacatcgccctgaacgaggacctgcgctcctggaccgccgcggacaccgcggctcagatcacccagcgcaagttggaggcggcccgtgcggcggagcagctgagagcctacctggagggcacgtgcgtggagtggctccgcagatacctggagaacgggaaggagacgctgcagcgcgcagaacccccaaagacacacgtgacccaccaccccctctctgaccatgaggccaccctgaggtgctgggccctgggcttctaccctgcggagatcacactgacctggcagcgggatggggaggaccagacccaggacaccgagcttgtggagaccaggccagcaggagatggaaccttccagaagtgggcagctgtggtggtgccttctggacaagagcagagatacacgtgccatatgcagcacgaggggctgcaagagcccctcaccctgagctgggagccatcttcccagcccaccatccccatcatgggcatcgttgctggcctggctgtcctggttgtcctagctgtccttggagctgtggtcaccgctatgatgtgtaggaggaagagctcaggtggaaaaggagggagctgctctcaggctgcgtgcagcaacagtgcccagggctctgatgagtctctcatcacttgtaaagcctgagacagctgcctgtgtgggactgagatgcaggatttcttcacacctctcctttgtgacttcaagagcctctggcatctctttctgcaaaggcacctgaatgtgtctgcgttcctgttagcataatgtgaggaggtggagagacagcccacccccgtgtccaccgtgacccctgtccccacactgacctgtgttccctccccgatcatctttcctgttccagagaggtggggctggatgtctccatctctgtctcaaattcatggtgcactgagctgcaacttcttacttccctaatgaagttaagaacctgaatataaatttgtgttctcaaatatttgctatgaagcgttgatggattaattaaataagtcaattcctagaagttgagagagcaaataaagacctgagaaccttccagaa

SEQ ID NO: 8 - protein, 366 aa, Homo sapiens
MRVMAPRALLLLLSGGLALTETWACSHSMRYFDTAVSRPGRGEPRFISVGYVDDTQFVRFDSDAASPRGEPRAPWVEQEGPEYWDRETQKYKRQAQADRVSLRNLRGYYNQSEDGSHTLQRMSGCDLGPDGRLLRGYDQSAYDGKDYIALNEDLRSWTAADTAAQITQRKLEAARAAEQLRAYLEGTCVEWLRRYLENGKETLQRAEPPKTHVTHHPLSDHEATLRCWALGFYPAEITLTWQRDGEDQTQDTELVETRPAGDGTFQKWAAVVVPSGQEQRYTCHMQHEGLQEPLTLSWEPSSQPTIPIMGIVAGLAVLVVLAVLGAVVTAMMCRRKSSGGKGGSCSQAACSNSAQGSDESLITCKA

SEQ ID NO: 9 - DNA, 2679 bp, Homo sapiens
  CDS (127)..(1203)
gcagactcagttctcattcccaatgggtgtcgggtttctagagaagccaatcagcgtcgccacgactcccgactataaagtccccatccggactcaagaagttctcaggactcagaggctgggatcatggtagatggaaccctccttttactcctctcggaggccctggcccttacccagacctgggcgggctcccactccttgaagtatttccacacttccgtgtcccggcccggccgcggggagccccgcttcatctctgtgggctacgtggacgacacccagttcgtgcgcttcgacaacgacgccgcgagtccgaggatggtgccgcgggcgccgtggatggagcaggaggggtcagagtattgggaccgggagacacggagcgccagggacaccgcacagattttccgagtgaatctgcggacgctgcgcggctactacaatcagagcgaggccgggtctcacaccctgcagtggatgcatggctgcgagctggggcccgacgggcgcttcctccgcgggtatgaacagttcgcctacgacggcaaggattatctcaccctgaatgaggacctgcgctcctggaccgcggtggacacggcggctcagatctccgagcaaaagtcaaatgatgcctctgaggcggagcaccagagagcctacctggaagacacatgcgtggagtggctccacaaatacctggagaaggggaaggagacgctgcttcacctggagcccccaaagacacacgtgactcaccaccccatctctgaccatgaggccaccctgaggtgctgggccctgggcttctaccctgcggagatcacactgacctggcagcaggatggggagggccatacccaggacacggagctcgtggagaccaggcctgcaggggatggaaccttccagaagtgggcagctgtggtggtgccttctggagaggagcagagatacacgtgccatgtgcagcatgaggggctacccgagcccgtcaccctgagatggaagccggcttcccagcccaccatccccatcgtgggcatcattgctggcctggttctccttggatctgtggtctctggagctgtggttgctgctgtgatatggaggaagaagagctcaggtggaaaaggagggagctactctaaggctgagtggagcgacagtgcccaggggtctgagtctcacagcttgtaaagcctgagacagctgccttgtgtgcgactgagatgcacagctgccttgtgtgcgactgagatgcaggatttcctcacgcctcccctatgtgtcttaggggactctggcttctctttttgcaagggcctctgaatctgtctgtgtccctgttagcacaatgtgaggaggtagagaaacagtccacctctgtgtctaccatgacccccttcctcacactgacctgtgttccttccctgttctcttttctattaaaaataagaacctgggcagagtgcggcagctcatgcctgtaatcccagcacttagggaggccgaggagggcagatcacgaggtcaggagatcgaaaccatcctggctaacacggtgaaaccccgtctctactaaaaaatacaaaaaattagctgggcgcagaggcacgggcctgtagtcccagctactcaggaggcggaggcaggagaatggcgtcaacccgggaggcggaggttgcagtgagccaggattgtgcgactgcactccagcctgggtgacagggtgaaacgccatctcaaaaaataaaaattgaaaaataaaaaaagaacctggatctcaatttaatttttcatattcttgcaatgaaatggacttgaggaagctaagatcatagctagaaatacagataattccacagcacatctctagcaaatttagcctattcctattctctagcctattccttaccacctgtaatcttgaccatataccttggagttgaatattgttttcatactgctgtggtttgaatgttccctccaacactcatgttgagacttaatccctaatgtggcaatactgaaaggtggggcctttgagatgtgattggatcgtaaggctgtgccttcattcatgggttaatggattaatgggttatcacaggaatgggactggtggctttataagaagaggaaaagagaactgagctagcatgcccagcccacagagagcctccactagagtgatgctaagtggaaatgtgaggtgcagctgccacagagggcccccaccagggaaatgtctagtgtctagtggatccaggccacaggagagagtgccttgtggagcgctgggagcaggacctgaccaccaccaggaccccagaactgtggagtcagtggcagcatgcagcgcccccttgggaaagctttaggcaccagcctgcaacccattcgagcagccacgtaggctgcacccagcaaagccacaggcacggggctacctgaggccttgggggcccaatccctgctccagtgtgtccgtgaggcagcacacgaagtcaaaagagattattctcttcccacagataccttttctctcccatgaccctttaacagcatctgcttcattcccctcaccttcccaggctgatctgaggtaaactttgaagtaaaataaaagctgtgtttgagcatcatttgtatttcaaaaaaaaaaaaaaaaaa

SEQ ID NO: 10 - protein, 358 aa, Homo sapiens
MVDGTLLLLLSEALALTQTWAGSHSLKYFHTSVSRPGRGEPRFISVGYVDDTQFVRFDNDAASPRMVPRAPWMEQEGSEYWDRETRSARDTAQIFRVNLRTLRGYYNQSEAGSHTLQWMHGCELGPDGRFLRGYEQFAYDGKDYLTLNEDLRSWTAVDTAAQISEQKSNDASEAEHQRAYLEDTCVEWLHKYLEKGKETLLHLEPPKTHVTHHPISDHEATLRCWALGFYPAEITLTWQQDGEGHTQDTELVETRPAGDGTFQKWAAVVVPSGEEQRYTCHVQHEGLPEPVTLRWKPASQPTIPIVGIIAGLVLLGSVVSGAVVAAVIWRKKSSGGKGGSYSKAEWSDSAQGSESHSL

SEQ ID NO: 11 - DNA, 1301 bp, Homo sapiens
  CDS (125)..(1165)
tttctcactcccattgggcgtcgcgtttctagagaagccaatcagtgtcgccgcagttcccaggttctaaagtcccacgcaccccgcgggactcatatttttcccagacgcggaggttggggtcatggcgccccgaagcctcctcctgctgctctcaggggccctggccctgaccgatacttgggcgggctcccactccttgaggtatttcagcaccgctgtgtcgcggcccggccgcggggagccccgctacatcgccgtggagtacgtagacgacacgcaattcctgcggttcgacagcgacgccgcgattccgaggatggagccgcgggagccgtgggtggagcaagaggggccgcagtattgggagtggaccacagggtacgccaaggccaacgcacagactgaccgagtggccctgaggaacctgctccgccgctacaaccagagcgaggctgggtctcacaccctccagggaatgaatggctgcgacatggggcccgacggacgcctcctccgcgggtatcaccagcacgcgtacgacggcaaggattacatctccctgaacgaggacctgcgctcctggaccgcggcggacaccgtggctcagatcacccagcgcttctatgaggcagaggaatatgcagaggagttcaggacctacctggagggcgagtgcctggagttgctccgcagatacttggagaatgggaaggagacgctacagcgcgcagatcctccaaaggcacacgttgcccaccaccccatctctgaccatgaggccaccctgaggtgctgggccctgggcttctaccctgcggagatcacgctgacctggcagcgggatggggaggaacagacccaggacacagagcttgtggagaccaggcctgcaggggatggaaccttccagaagtgggccgctgtggtggtgcctcctggagaggaacagagatacacatgccatgtgcagcacgaggggctgccccagcccctcatcctgagatgggagcagtctccccagcccaccatccccatcgtgggcatcgttgctggccttgttgtccttggagctgtggtcactggagctgtggtcgctgctgtgatgtggaggaagaagagctcagatagaaacagagggagctactctcaggctgcagtgtgagacagcttccttgtgtgggactgagaagcaagatatcaatgtagcagaattgcacttgtgcctcacgaacatacataaattttaaaaataaagaataaaaatatatctttttatagataaaaaaaaaaaaaaaaaa

SEQ ID NO: 12 - protein, 346 aa, Homo sapiens
MAPRSLLLLLSGALALTDTWAGSHSLRYFSTAVSRPGRGEPRYIAVEYVDDTQFLRFDSDAAIPRMEPREPWVEQEGPQYWEWTTGYAKANAQTDRVALRNLLRRYNQSEAGSHTLQGMNGCDMGPDGRLLRGYHQHAYDGKDYISLNEDLRSWTAADTVAQITQRFYEAEEYAEEFRTYLEGECLELLRRYLENGKETLQRADPPKAHVAHHPISDHEATLRCWALGFYPAEITLTWQRDGEEQTQDTELVETRPAGDGTFQKWAAVVVPPGEEQRYTCHVQHEGLPQPLILRWEQSPQPTIPIVGIVAGLVVLGAVVTGAVVAAVMWRKKSSDRNRGSYSQAAV

SEQ ID NO: 13 - DNA, 1578 bp, Homo sapiens
  CDS (179)..(1195)
agtgtggtactttgtcttgaggagatgtcctggactcacacggaaacttagggctacggaatgaagttctcactcccattaggtgacaggtttttagagaagccaatcagcgtcgccgcggtcctggttctaaagtcctcgctcacccacccggactcattctccccagacgccaaggatggtggtcatggcgccccgaaccctcttcctgctgctctcgggggccctgaccctgaccgagacctgggcgggctcccactccatgaggtatttcagcgccgccgtgtcccggcccggccgcggggagccccgcttcatcgccatgggctacgtggacgacacgcagttcgtgcggttcgacagcgactcggcgtgtccgaggatggagccgcgggcgccgtgggtggagcaggaggggccggagtattgggaagaggagacacggaacaccaaggcccacgcacagactgacagaatgaacctgcagaccctgcgcggctactacaaccagagcgaggccagttctcacaccctccagtggatgattggctgcgacctggggtccgacggacgcctcctccgcgggtatgaacagtatgcctacgatggcaaggattacctcgccctgaacgaggacctgcgctcctggaccgcagcggacactgcggctcagatctccaagcgcaagtgtgaggcggccaatgtggctgaacaaaggagagcctacctggagggcacgtgcgtggagtggctccacagatacctggagaacgggaaggagatgctgcagcgcgcggacccccccaagacacacgtgacccaccaccctgtctttgactatgaggccaccctgaggtgctgggccctgggcttctaccctgcggagatcatactgacctggcagcgggatggggaggaccagacccaggacgtggagctcgtggagaccaggcctgcaggggatggaaccttccagaagtgggcagctgtggtggtgccttctggagaggagcagagatacacgtgccatgtgcagcatgaggggctgccggagcccctcatgctgagatggaagcagtcttccctgcccaccatccccatcatgggtatcgttgctggcctggttgtccttgcagctgtagtcactggagctgcggtcgctgctgtgctgtggagaaagaagagctcagattgaaaaggagggagctactctcaggctgcaatgtgaaacagctgccctgtgtgggactgagtggcaagtccctttgtgacttcaagaaccctgactcctctttgtgcagagaccagcccacccctgtgcccaccatgaccctcttcctcatgctgaactgcattccttccccaatcacctttcctgttccagaaaaggggctgggatgtctccgtctctgtctcaaatttgtggtccactgagctataacttacttctgtattaaaattagaatctgagtataaatttactttttcaaattatttccaagagagattgatgggttaattaaaggagaagattcctgaaatttgagagacaaaataaatggaagacatgagaacttt

SEQ ID NO: 14 - protein, 338 aa, Homo sapiens
MVVMAPRTLFLLLSGALTLTETWAGSHSMRYFSAAVSRPGRGEPRFIAMGYVDDTQFVRFDSDSACPRMEPRAPWVEQEGPEYWEEETRNTKAHAQTDRMNLQTLRGYYNQSEASSHTLQWMIGCDLGSDGRLLRGYEQYAYDGKDYLALNEDLRSWTAADTAAQISKRKCEAANVAEQRRAYLEGTCVEWLHRYLENGKEMLQRADPPKTHVTHHPVFDYEATLRCWALGFYPAEIILTWQRDGEDQTQDVELVETRPAGDGTFQKWAAVVVPSGEEQRYTCHVQHEGLPEPLMLRWKQSSLPTIPIMGIVAGLVVLAAVVTGAAVAAVLWRKKSSD

SEQ ID NO: 15 - DNA, 9232 bp, Artificial Sequence
  Vector sequence for human B2M-HLA-A0201 fusion protein
ctcgaggagcttggcccattgcatacgttgtatccatatcataatatgtacatttatattggctcatgtccaacattaccgccatgttgacattgattattgactagttattaatagtaatcaattacggggtcattagttcatagcccatatatggagttccgcgttacataacttacggtaaatggcccgcctggctgaccgcccaacgacccccgcccattgacgtcaataatgacgtatgttcccatagtaacgccaatagggactttccattgacgtcaatgggtggagtatttacgctaaactgcccacttggcagtacatcaagtgtatcatatgccaagtacgccccctattgacgtcaatgacggtaaatggcccgcctggcattatgcccagtacatgaccttatgggactttcctacttggcagtacatctacgtattagtcatcgctattaccatggtgatgcggttttggcagtacatcaatgggcgtggatagcggtttgactcacggggatttccaagtctccaccccattgacgtcaatgggagtttgttttggcaccaaaatcaacgggactttccaaaatgtcgtaacaactccgccccattgacgcaaatgggcggtaggcgtgtacggtgggaggtctatataagcagagcttctagattgtacgggagctcttcactactcgctgcgtcgagagtgtacgagactctccaggtttggtaagaaatattttatattgttataatgttactatgatccattaacactctgcttatagattgtaagggtgattgcaatgctttctgcataaaactttggttttcttgttaatcaataaaccgacttgattcgagaacctactcatatattattgtctcttttatactttattaagtaaaaggatttgtatattagccttgctaagggagacatctagtgatataagtgtgaactacacttatcttaaatgatgtaactccttaggataatcaatatacaaaattccatgacaattggcgcccaacgtggggctcgaatataagtcgggtttatttgtaaattatccctagggacctccgagcaagcgagcatagcgggaggcatataaaagccaatagacaatggctagcaggaagtaatgttgaagaatatgaacttgatgttgaagctctggttgtaattttaagagatagaaatataccaagaaatcctttacatggagaagttataggtcttcgccttactgaaggatggtggggacaaattgagagatttcagatggtacgttgatctaaggctatggatttggccatgggacaagaaatattagtttatagtcccattgtatctatgactaaaatacaaaaaactccactaccagaaagaaaagctttacccattagatggataacatggatgacttatttagaagatccaagaatccaatttcattatgataaaaccttaccagaacttaagcatattccagatgtatatacatctagtcagtctcctgttaaacatccttctcaatatgaaggagtgttttatactgatggctcggccatcaaaagtcctgatcctacaaaaagcaataatgctggcatgggaatagtacatgccacatacaaacctgaatatcaagttttgaatcaatggtcaataccactaggtaatcatactgctcagatggctgaaatagctgcagttgaatttgcctgtaaaaaagctttaaaaatacctggtcctgtattagttataactgatagtttctatgtagcagaaagtgctaataaagaattaccatactggaaatctaatgggtttgttaataataagaaaaagcctcttaaacatatctccaaatggaaatctattgctgagtgtttatctatgaaaccagacattactattcaacatgaaaaaggcatcagcctacaaataccagtattcatactgaaaggcaatgccctagcagataagcttgccacccaaggaagttatgtggttaattgtaataccaaaaaaccaaacctggatgcagagttggatcaattattacagggtcattatataaaaggatatcccaaacaatatacatattttttagaagatggcaaagtaaaagtttccagacctgaaggggttaaaattattccccctcagtcagacagacaaaaaattgtgcttcaagcccacaatttggctcacaccggacgtgaagccactcttttaaaaattgccaacctttattggtggccaaatatgagaaaggatgtggttaaacaactaggacgctgtcaacagtgtttaatcacaaatgcttccaacaaagcctctggtcctattctaagaccagataggcctcaaaaaccttttgataaattctttattgactatattggacctttgccaccttcacagggatacctatatgtattagtagttgttgatggaatgacaggattcacttggttataccccactaaggctccttctactagcgcaactgttaaatctctcaatgtactcactagtattgcaattccaaaggtgattcactctgatcaaggtgcagcattcacttcttcaacctttgctgaatgggcaaaggaaagaggtatacatttggaattcagtactccttatcacccccaaagtggtagtaaggtggaaaggaaaaatagtgatataaaacgacttttaactaaactgctagtaggaagacccacaaagtggtatgacctattgcctgttgtacaacttgctttaaacaacacctatagccctgtattaaaatatactccacatcaactcttatttggtatagattcaaatactccatttgcaaatcaagatacacttgacttgaccagagaagaagaactttctcttttacaggaaattcgtacttctttataccatccatccacccctccagcctcctctcgttcctggtctcctgttgttggccaattggtccaggagagggtggctaggcctgcttctttgagacctcgttggcataaaccgtctactgtacttaaggtgttgaatccaaggactgttgttattttggaccatcttggcaacaacagaactgtaagtatagataatttaaaacctacttctcatcagaatggcaccaccaatgacactgcaacaatggatcatttggaaaaaaatgaataaagcgcatgaggcacttcaaaatacaacaactgtgactgaacagcagaaggaacaaattatactggacattcaaaatgaagaagtacaaccaactaggagagataaatttagatatctgctttatacttgttgtgctactagctcaagagtattggcctggatgtttttagtttgtatattgttaatcattgttttggtttcatgctttgtgactatatccagaatacaatggaataaggatattcaggtattaggacctgtaatagactggaatgttactcaaagagctgtttatcaacccttacagactagaaggattgcacgttcccttagaatgcagcatcctgttccaaaatatgtggaggtaaatatgactagtattccacaaggtgtatactatgaaccccatccggcctcgacggtatcgatggtaccggtatcgataagcttgataacctcgagagatctaattctaccgggtaggggaggcgcttttcccaaggcagtctggagcatgcgctttagcagccccgctggcacttggcgctacacaagtggcctctggcctcgcacacattccacatccaccggtagcgccaaccggctccgttctttggtggccccttcgcgccacttctactcctcccctagtcaggaagtttcccccagcaagctcgcgtcgtgcaggacgtgacaaatggaagtagcacgtctcactagtctcgtgcagatggacagcaccgctgagcaatggaagcgggtaggcctttggggcagcggccaatagcagctttgttccttcgctttctgggctcagaggctgggaaggggtgggtccgggggcgggctcaggggcgggctcaggggcgggcgggcgcccgaaggtcctcccgaggcccggcattctgcacgcttcaaaagcgcacgtctgccgcgctgttctcctcttcctcatctccgggcctttcgacctgcagcccgggggatcgatcctaggtgatttaaatccaccatgaccgagtacaagcccacggtgcgcctcgccacccgcgacgacgtcccccgggccgtacgcaccctcgccgccgcgttcgccgactaccccgccacgcgccacaccgtcgacccggaccgccacatcgagcgggtcaccgagctgcaagaactcttcctcacgcgcgtcgggctcgacatcggcaaggtgtgggtcgcggacgacggcgccgcggtggcggtctggaccacgccggagagcgtcgaagcgggggcggtgttcgccgagatcggcccgcgcatggccgagttgagcggttcccggctggccgcgcagcaacagatggaaggcctcctggcgccgcaccggcccaaggagcccgcgtggttcctggccaccgtcggcgtctcgcccgaccaccagggcaagggtctgggcagcgccgtcgtgctccccggagtggaggcggccgagcgcgccggggtgcccgccttcctggagacctccgcgccccgcaacctccccttctacgagcggctcggcttcaccgtcaccgccgacgtcgagtgcccgaaggaccgcgcgacctggtgcatgacccgcaagcccggtgcctgacggatccatcgctccggtgcccgtcagtgggcagagcgcacatcgcccacagtccccgagaagttggggggaggggtcggcaattgaaccggtgcctagagaaggtggcgcggggtaaactgggaaagtgatgtcgtgtactggctccgcctttttcccgagggtgggggagaaccgtatataagtgcagtagtcgccgtgaacgttctttttcgcaacgggtttgccgccagaacacagctgcggccgcgccgccaccatgtctcgctccgtggccttagctgtgctcgcgctactctctctttctggcctggaggctatccagcgtactccaaagattcaggtttactcacgtcatccagcagagaatggaaagtcaaatttcctgaattgctatgtgtctgggtttcatccatccgacattgaagttgacttactgaagaatggagagagaattgaaaaagtggagcattcagacttgtctttcagcaaggactggtctttctatctcttgtactacactgaattcacccccactgaaaaagatgagtatgcctgccgtgtgaaccatgtgactttgtcacagcccaagatagttaagtgggatcgagacatgggcggaggcggaagcgggggcggcggatccggcggaggcggaagcggcggcgggggaagcggctctcactccatgaggtatttcttcacatccgtgtcccggcccggccgcggggagccccgcttcatcgcagtgggctacgtggacgacacgcagttcgtgcggttcgacagcgacgccgcgagccagaggatggagccgcgggcgccgtggatagagcaggagggtccggagtattgggacggggagacacggaaagtgaaggcccactcacagactcaccgagtggacctggggaccctgcgcggctactacaaccagagcgaggccggttctcacaccgtccagaggatgtatggctgcgacgtggggtcggactggcgcttcctccgcgggtaccaccagtacgcctacgacggcaaggattacatcgccctgaaagaggacctgcgctcttggaccgcggcggacatggcagctcagaccaccaagcacaagtgggaggcggcccatgtggcggagcagttgagagcctacctggagggcacgtgcgtggagtggctccgcagatacctggagaacgggaaggagacgctgcagcgcacggacgcccccaaaacgcatatgactcaccacgctgtctctgaccatgaagccaccctgaggtgctgggccctgagcttctaccctgcggagatcacactgacctggcagcgggatggggaggaccagacccaggacacggagctcgtggagaccaggcctgcaggggatggaaccttccagaagtgggcggctgtggtggtgccttctggacaggagcagagatacacctgccatgtgcagcatgagggtttgcccaagcccctcaccctgagatgggagccgtcttcccagcccaccatccccatcgtgggcatcattgctggcctggttctctttggagctgtgatcactggagctgtggtcgctgctgtgatgtggaggaggaagagctcagatagaaaaggagggagctactctcaggctgcaagcagtgacagtgcccagggctctgatgtgtctctcacagcttgtaaagtgtgagcggccgcgactctagatcaggcgcgccgttaccaagcagctatggaagcttatggacctcagagaggaagtaacgaggagagggtgtggtggaatgtcactagaaaccagggaaaacaaggaggagagtattacagggaaggaggtgaagaacctcattacccaaatactcctgctcctcatagacgtacctgggatgagagacacaaggttcttaaattgtcctcattcgctactccctctgacatccaacgctgggctactaactctagattgtacgggagctctcttcactactcgctgcgtcgagagtgtacgagactctccaggtttggtaagaaatattttatattgttataatgttactatgatccattaacactctgcttatagattgtaagggtgattgcaatgctttctgcataaaactttggttttcttgttaatcaataaaccgacttgattcgagaacctactcatatattattgtctcttttatactttattaagtaaaaggatttgtatattagccttgctaagggagacatctagtgatataagtgtgaactacacttatcttaaatgatgtaactccttaggataatcaatatacaaaattccatgacaattggcgataccgtcgaccgttcagctgcattaatgaatcggccaacgcgcggggagaggcggtttgcgtattgggcgctcttccgcttcctcgctcactgactcgctgcgctcggtcgttcggctgcggcgagcggtatcagctcactcaaaggcggtaatacggttatccacagaatcaggggataacgcaggaaagaacatgtgagcaaaaggccagcaaaaggccaggaaccgtaaaaaggccgcgttgctggcgtttttccataggctccgcccccctgacgagcatcacaaaaatcgacgctcaagtcagaggtggcgaaacccgacaggactataaagataccaggcgtttccccctggaagctccctcgtgcgctctcctgttccgaccctgccgcttaccggatacctgtccgcctttctcccttcgggaagcgtggcgctttctcaatgctcacgctgtaggtatctcagttcggtgtaggtcgttcgctccaagctgggctgtgtgcacgaaccccccgttcagcccgaccgctgcgccttatccggtaactatcgtcttgagtccaacccggtaagacacgacttatcgccactggcagcagccactggtaacaggattagcagagcgaggtatgtaggcggtgctacagagttcttgaagtggtggcctaactacggctacactagaaggacagtatttggtatctgcgctctgctgaagccagttaccttcggaaaaagagttggtagctcttgatccggcaaacaaaccaccgctggtagcggtggtttttttgtttgcaagcagcagattacgcgcagaaaaaaaggatctcaagaagatcctttgatcttttctacggggtctgacgctcagtggaacgaaaactcacgttaagggattttggtcatgagattatcaaaaaggatcttcacctagatccttttaaattaaaaatgaagttttaaatcaatctaaagtatatatgagtaaacttggtctgacagttaccaatgcttaatcagtgaggcacctatctcagcgatctgtctatttcgttcatccatagttgcctgactccccgtcgtgtagataactacgatacgggagggcttaccatctggccccagtgctgcaatgataccgcgagacccacgctcaccggctccagatttatcagcaataaaccagccagccggaagggccgagcgcagaagtggtcctgcaactttatccgcctccatccagtctattaattgttgccgggaagctagagtaagtagttcgccagttaatagtttgcgcaacgttgttgccattgctacaggcatcgtggtgtcacgctcgtcgtttggtatggcttcattcagctccggttcccaacgatcaaggcgagttacatgatcccccatgttgtgcaaaaaagcggttagctccttcggtcctccgatcgttgtcagaagtaagttggccgcagtgttatcactcatggttatggcagcactgcataattctcttactgtcatgccatccgtaagatgcttttctgtgactggtgagtactcaaccaagtcattctgagaatagtgtatgcggcgaccgagttgctcttgcccggcgtcaatacgggataataccgcgccacatagcagaactttaaaagtgctcatcattggaaaacgttcttcggggcgaaaactctcaaggatcttaccgctgttgagatccagttcgatgtaacccactcgtgcacccaactgatcttcagcatcttttactttcaccagcgtttctgggtgagcaaaaacaggaaggcaaaatgccgcaaaaaagggaataagggcgacacggaaatgttgaatactcatactcttcctttttcaatattattgaagcatttatcagggttattgtctcatgagcggatacatatttgaatgtatttagaaaaataaacaaataggggttccgcgcacatttccccgaaaagtgccacctgacgtctaagaaaccattattatcatgacattaacctataaaaataggcgtatcacgaggccctttcgtc

SEQ ID NO: 16 - protein, 480 aa, Artificial Sequence
  HLA-bBA0201 (human B2M-HLA-A0201 fusion peptide)
MSRSVALAVLALLSLSGLEAIQRTPKIQVYSRHPAENGKSNFLNCYVSGFHPSDIEVDLLKNGERIEKVEHSDLSFSKDWSFYLLYYTEFTPTEKDEYACRVNHVTLSQPKIVKWDRDMGGGGSGGGGSGGGGSGGGGSGSHSMRYFFTSVSRPGRGEPRFIAVGYVDDTQFVRFDSDAASQRMEPRAPWIEQEGPEYWDGETRKVKAHSQTHRVDLGTLRGYYNQSEAGSHTVQRMYGCDVGSDWRFLRGYHQYAYDGKDYIALKEDLRSWTAADMAAQTTKHKWEAAHVAEQLRAYLEGTCVEWLRRYLENGKETLQRTDAPKTHMTHHAVSDHEATLRCWALSFYPAEITLTWQRDGEDQTQDTELVETRPAGDGTFQKWAAVVVPSGQEQRYTCHVQHEGLPKPLTLRWEPSSQPTIPIVGIIAGLVLFGAVITGAVVAAVMWRRKSSDRKGGSYSQAASSDSAQGSDVSLTACKV

SEQ ID NO: 17 - DNA, 9224 bp, Artificial Sequence
  Vector sequence for HLA-gBE
ctcgaggagcttggcccattgcatacgttgtatccatatcataatatgtacatttatattggctcatgtccaacattaccgccatgttgacattgattattgactagttattaatagtaatcaattacggggtcattagttcatagcccatatatggagttccgcgttacataacttacggtaaatggcccgcctggctgaccgcccaacgacccccgcccattgacgtcaataatgacgtatgttcccatagtaacgccaatagggactttccattgacgtcaatgggtggagtatttacgctaaactgcccacttggcagtacatcaagtgtatcatatgccaagtacgccccctattgacgtcaatgacggtaaatggcccgcctggcattatgcccagtacatgaccttatgggactttcctacttggcagtacatctacgtattagtcatcgctattaccatggtgatgcggttttggcagtacatcaatgggcgtggatagcggtttgactcacggggatttccaagtctccaccccattgacgtcaatgggagtttgttttggcaccaaaatcaacgggactttccaaaatgtcgtaacaactccgccccattgacgcaaatgggcggtaggcgtgtacggtgggaggtctatataagcagagcttctagattgtacgggagctcttcactactcgctgcgtcgagagtgtacgagactctccaggtttggtaagaaatattttatattgttataatgttactatgatccattaacactctgcttatagattgtaagggtgattgcaatgctttctgcataaaactttggttttcttgttaatcaataaaccgacttgattcgagaacctactcatatattattgtctcttttatactttattaagtaaaaggatttgtatattagccttgctaagggagacatctagtgatataagtgtgaactacacttatcttaaatgatgtaactccttaggataatcaatatacaaaattccatgacaattggcgcccaacgtggggctcgaatataagtcgggtttatttgtaaattatccctagggacctccgagcatagcgggaggcatataaaagccaatagacaatggctagcaggaagtaatgttgaagaatatgaacttgatgttgaagctctggttgtaattttaagagatagaaatataccaagaaatcctttacatggagaagttataggtcttcgccttactgaaggatggtggggacaaattgagagatttcagatggtacgttgatctaaggctatggatttggccatgggacaagaaatattagtttatagtcccattgtatctatgactaaaatacaaaaaactccactaccagaaagaaaagctttacccattagatggataacatggatgacttatttagaagatccaagaatccaatttcattatgataaaaccttaccagaacttaagcatattccagatgtatatacatctagtcagtctcctgttaaacatccttctcaatatgaaggagtgttttatactgatggctcggccatcaaaagtcctgatcctacaaaaagcaataatgctggcatgggaatagtacatgccacatacaaacctgaatatcaagttttgaatcaatggtcaataccactaggtaatcatactgctcagatggctgaaatagctgcagttgaatttgcctgtaaaaaagctttaaaaatacctggtcctgtattagttataactgatagtttctatgtagcagaaagtgctaataaagaattaccatactggaaatctaatgggtttgttaataataagaaaaagcctcttaaacatatctccaaatggaaatctattgctgagtgtttatctatgaaaccagacattactattcaacatgaaaaaggcatcagcctacaaataccagtattcatactgaaaggcaatgccctagcagataagcttgccacccaaggaagttatgtggttaattgtaataccaaaaaaccaaacctggatgcagagttggatcaattattacagggtcattatataaaaggatatcccaaacaatatacatattttttagaagatggcaaagtaaaagtttccagacctgaaggggttaaaattattccccctcagtcagacagacaaaaaattgtgcttcaagcccacaatttggctcacaccggacgtgaagccactcttttaaaaattgccaacctttattggtggccaaatatgagaaaggatgtggttaaacaactaggacgctgtcaacagtgtttaatcacaaatgcttccaacaaagcctctggtcctattctaagaccagataggcctcaaaaaccttttgataaattctttattgactatattggacctttgccaccttcacagggatacctatatgtattagtagttgttgatggaatgacaggattcacttggttataccccactaaggctccttctactagcgcaactgttaaatctctcaatgtactcactagtattgcaattccaaaggtgattcactctgatcaaggtgcagcattcacttcttcaacctttgctgaatgggcaaaggaaagaggtatacatttggaattcagtactccttatcacccccaaagtggtagtaaggtggaaaggaaaaatagtgatataaaacgacttttaactaaactgctagtaggaagacccacaaagtggtatgacctattgcctgttgtacaacttgctttaaacaacacctatagccctgtattaaaatatactccacatcaactcttatttggtatagattcaaatactccatttgcaaatcaagatacacttgacttgaccagagaagaagaactttctcttttacaggaaattcgtacttctttataccatccatccacccctccagcctcctctcgttcctggtctcctgttgttggccaattggtccaggagagggtggctaggcctgcttctttgagacctcgttggcataaaccgtctactgtacttaaggtgttgaatccaaggactgttgttattttggaccatcttggcaacaacagaactgtaagtatagataatttaaaacctacttctcatcagaatggcaccaccaatgacactgcaacaatggatcatttggaaaaaaatgaataaagcgcatgaggcacttcaaaatacaacaactgtgactgaacagcagaaggaacaaattatactggacattcaaaatgaagaagtacaaccaactaggagagataaatttagatatctgctttatacttgttgtgctactagctcaagagtattggcctggatgtttttagtttgtatattgttaatcattgttttggtttcatgctttgtgactatatccagaatacaatggaataaggatattcaggtattaggacctgtaatagactggaatgttactcaaagagctgtttatcaacccttacagactagaaggattgcacgttcccttagaatgcagcatcctgttccaaaatatgtggaggtaaatatgactagtattccacaaggtgtatactatgaaccccatccggcctcgacggtatcgatggtaccggtatcgataagcttgataacctcgagagatctaattctaccgggtaggggaggcgcttttcccaaggcagtctggagcatgcgctttagcagccccgctggcacttggcgctacacaagtggcctctggcctcgcacacattccacatccaccggtagcgccaaccggctccgttctttggtggccccttcgcgccacttctactcctcccctagtcaggaagtttcccccagcaagctcgcgtcgtgcaggacgtgacaaatggaagtagcacgtctcactagtctcgtgcagatggacagcaccgctgagcaatggaagcgggtaggcctttggggcagcggccaatagcagctttgttccttcgctttctgggctcagaggctgggaaggggtgggtccgggggcgggctcaggggcgggctcaggggcgggcgggcgcccgaaggtcctcccgaggcccggcattctgcacgcttcaaaagcgcacgtctgccgcgctgttctcctcttcctcatctccgggcctttcgacctgcagcccgggggatcgatcctaggtgatttaaatccaccatgaccgagtacaagcccacggtgcgcctcgccacccgcgacgacgtcccccgggccgtacgcaccctcgccgccgcgttcgccgactaccccgccacgcgccacaccgtcgacccggaccgccacatcgagcgggtcaccgagctgcaagaactcttcctcacgcgcgtcgggctcgacatcggcaaggtgtgggtcgcggacgacggcgccgcggtggcggtctggaccacgccggagagcgtcgaagcgggggcggtgttcgccgagatcggcccgcgcatggccgagttgagcggttcccggctggccgcgcagcaacagatggaaggcctcctggcgccgcaccggcccaaggagcccgcgtggttcctggccaccgtcggcgtctcgcccgaccaccagggcaagggtctgggcagcgccgtcgtgctccccggagtggaggcggccgagcgcgccggggtgcccgccttcctggagacctccgcgccccgcaacctccccttctacgagcggctcggcttcaccgtcaccgccgacgtcgagtgcccgaaggaccgcgcgacctggtgcatgacccgcaagcccggtgcctgacggatccatcgctccggtgcccgtcagtgggcagagcgcacatcgcccacagtccccgagaagttggggggaggggtcggcaattgaaccggtgcctagagaaggtggcgcggggtaaactgggaaagtgatgtcgtgtactggctccgcctttttcccgagggtgggggagaaccgtatataagtgcagtagtcgccgtgaacgttctttttcgcaacgggtttgccgccagaacacagctgcggccgcgttaaccatggtggtcatggcccctcgaactctgttcctgctgctgagtggggctctgaccctgacagagtccggaatccagcggacccccaagattcaggtgtacagcagacaccctgcagagaacggcaaatccaacttcctgaattgctatgtgtctgggtttcatcccagtgacatcgaagtcgatctgctgaagaatggcgagagaattgaaaaagtcgagcactctgacctgagcttctccaaggattggtccttttacctgctgtactataccgagtttactccaaccgaaaaagacgagtatgcctgtagggtgaaccatgtcacactgagccagcccaagatcgtgaaatgggaccgcgatatgggcgggggaggctcagggggaggcgggagcggaggcgggggctccggcgggggaggatccggttctcactccttgaagtatttccacacttccgtgtcccggcccggccgcggggagccccgcttcatctctgtgggctacgtggacgacacccagttcgtgcgcttcgacaacgacgccgcgagtccgaggatggtgccgcgggcgccgtggatggagcaggaggggtcagagtattgggaccgggagacacggagcgccagggacaccgcacagattttccgagtgaatctgcggacgctgcgcggctactacaatcagagcgaggccgggtctcacaccctgcagtggatgcatggctgcgagctggggcccgacgggcgcttcctccgcgggtatgaacagttcgcctacgacggcaaggattatctcaccctgaatgaggacctgcgctcctggaccgcggtggacacggcggctcagatctccgagcaaaagtcaaatgatgcctctgaggcggagcaccagagagcctacctggaagacacatgcgtggagtggctccacaaatacctggagaaggggaaggagacgctgcttcacctggagcccccaaagacacacgtgactcaccaccccatctctgaccatgaggccaccctgaggtgctgggccctgggcttctaccctgcggagatcacactgacctggcagcaggatggggagggccatacccaggacacggagctcgtggagaccaggcctgcaggggatggaaccttccagaagtgggcagctgtggtggtgccttctggagaggagcagagatacacgtgccatgtgcagcatgaggggctacccgagcccgtcaccctgagatggaagccggcttcccagcccaccatccccatcgtgggcatcattgctggcctggttctccttggatctgtggtctctggagctgtggttgctgctgtgatatggaggaagaagagctcaggtggaaaaggagggagctactctaaggctgagtggagcgacagtgcccaggggtctgagtctcacagcttgtaatctagagcggccgcgactctagatcaggcgcgccgttaccaagcagctatggaagcttatggacctcagagaggaagtaacgaggagagggtgtggtggaatgtcactagaaaccagggaaaacaaggaggagagtattacagggaaggaggtgaagaacctcattacccaaatactcctgctcctcatagacgtacctgggatgagagacacaaggttcttaaattgtcctcattcgctactccctctgacatccaacgctggactactaactctagattgtacgggaggctcttcactactcgctgcgtcgagagtgtacgagactctccaggtttggtaagaaatattttatattgttataatgttactatgatccattaacactctgcttatagattgtaagggtgattgcaatgctttctgcataaaactttggttttcttgttaatcaataaaccgacttgattcgagaaccaactcctatattattgtctcttttatactttattaagtaaaaggatttgtatattagccttgctaagggagacatctagtgatataagtgtgaactacacttatcttaaatgatgtaactccttaggataatcaatatacaaaattccatgacaattggcgataccgtcgaccgttcagctgcattaatgaatcggccaacgcgcggggagaggcggtttgcgtattgggcgctcttccgcttcctcgctcactgactcgctgcgctcggtcgttcggctgcggcgagcggtatcagctcactcaaaggcggtaatacggttatccacagaatcaggggataacgcaggaaagaacatgtgagcaaaaggccagcaaaaggccaggaaccgtaaaaaggccgcgttgctggcgtttttccataggctccgcccccctgacgagcatcacaaaaatcgacgctcaagtcagaggtggcgaaacccgacaggactataaagataccaggcgtttccccctggaagctccctcgtgcgctctcctgttccgaccctgccgcttaccggatacctgtccgcctttctcccttcgggaagcgtggcgctttctcaatgctcacgctgtaggtatctcagttcggtgtaggtcgttcgctccaagctgggctgtgtgcacgaaccccccgttcagcccgaccgctgcgccttatccggtaactatcgtcttgagtccaacccggtaagacacgacttatcgccactggcagcagccactggtaacaggattagcagagcgaggtatgtaggcggtgctacagagttcttgaagtggtggcctaactacggctacactagaaggacagtatttggtatctgcgctctgctgaagccagttaccttcggaaaaagagttggtagctcttgatccggcaaacaaaccaccgctggtagcggtggtttttttgtttgcaagcagcagattacgcgcagaaaaaaaggatctcaagaagatcctttgatcttttctacggggtctgacgctcagtggaacgaaaactcacgttaagggattttggtcatgagattatcaaaaaggatcttcacctagatccttttaaattaaaaatgaagttttaaatcaatctaaagtatatatgagtaaacttggtctgacagttaccaatgcttaatcagtgaggcacctatctcagcgatctgtctatttcgttcatccatagttgcctgactccccgtcgtgtagataactacgatacgggagggcttaccatctggccccagtgctgcaatgataccgcgagacccacgctcaccggctccagatttatcagcaataaaccagccagccggaagggccgagcgcagaagtggtcctgcaactttatccgcctccatccagtctattaattgttgccgggaagctagagtaagtagttcgccagttaatagtttgcgcaacgttgttgccattgctacaggcatcgtggtgtcacgctcgtcgtttggtatggcttcattcagctccggttcccaacgatcaaggcgagttacatgatcccccatgttgtgcaaaaaagcggttagctccttcggtcctccgatcgttgtcagaagtaagttggccgcagtgttatcactcatggttatggcagcactgcataattctcttactgtcatgccatccgtaagatgcttttctgtgactggtgagtactcaaccaagtcattctgagaatagtgtatgcggcgaccgagttgctcttgcccggcgtcaatacgggataataccgcgccacatagcagaactttaaaagtgctcatcattggaaaacgttcttcggggcgaaaactctcaaggatcttaccgctgttgagatccagttcgatgtaacccactcgtgcacccaactgatcttcagcatcttttactttcaccagcgtttctgggtgagcaaaaacaggaaggcaaaatgccgcaaaaaagggaataagggcgacacggaaatgttgaatactcatactcttcctttttcaatattattgaagcatttatcagggttattgtctcatgagcggatacatatttgaatgtatttagaaaaataaacaaataggggttccgcgcacatttccccgaaaagtgccacctgacgtctaagaaaccattattatcatgacattaacctataaaaataggcgtatcacgaggccctttcgtc

SEQ ID NO: 18 - protein, 476 aa, Artificial Sequence
  HLA-gBE
MAPRTLFLLLSGALTLTESGIQRTPKIQVYSRHPAENGKSNFLNCYVSGFHPSDIEVDLLKNGERIEKVEHSDLSFSKDWSFYLLYYTEFTPTEKDEYACRVNHVTLSQPKIVKWDRDMGGGGSGGGGSGGGGSGGGGSGSHSLKYFHTSVSRPGRGEPRFISVGYVDDTQFVRFDNDAASPRMVPRAPWMEQEGSEYWDRETRSARDTAQIFRVNLRTLRGYYNQSEAGSHTLQWMHGCELGPDGRFLRGYEQFAYDGKDYLTLNEDLRSWTAVDTAAQISEQKSNDASEAEHQRAYLEDTCVEWLHKYLEKGKETLLHLEPPKTHVTHHPISDHEATLRCWALGFYPAEITLTWQQDGEGHTQDTELVETRPAGDGTFQKWAAVVVPSGEEQRYTCHVQHEGLPEPVTLRWKPASQPTIPIVGIIAGLVLLGSVVSGAVVAAVIWRKKSSGGKGGSYSKAEWSDSAQGSESHSL

SEQ ID NO: 19 - DNA, 9287 bp, Artificial Sequence
  Vector sequence for HLA-bGBE
ctcgaggagcttggcccattgcatacgttgtatccatatcataatatgtacatttatattggctcatgtccaacattaccgccatgttgacattgattattgactagttattaatagtaatcaattacggggtcattagttcatagcccatatatggagttccgcgttacataacttacggtaaatggcccgcctggctgaccgcccaacgacccccgcccattgacgtcaataatgacgtatgttcccatagtaacgccaatagggactttccattgacgtcaatgggtggagtatttacgctaaactgcccacttggcagtacatcaagtgtatcatatgccaagtacgccccctattgacgtcaatgacggtaaatggcccgcctggcattatgcccagtacatgaccttatgggactttcctacttggcagtacatctacgtattagtcatcgctattaccatggtgatgcggttttggcagtacatcaatgggcgtggatagcggtttgactcacggggatttccaagtctccaccccattgacgtcaatgggagtttgttttggcaccaaaatcaacgggactttccaaaatgtcgtaacaactccgccccattgacgcaaatgggcggtaggcgtgtacggtgggaggtctatataagcagagcttctagattgtacgggagctcttcactactcgctgcgtcgagagtgtacgagactctccaggtttggtaagaaatattttatattgttataatgttactatgatccattaacactctgcttatagattgtaagggtgattgcaatgctttctgcataaaactttggttttcttgttaatcaataaaccgacttgattcgagaacctactcatatattattgtctcttttatactttattaagtaaaaggatttgtatattagccttgctaagggagacatctagtgatataagtgtgaactacacttatcttaaatgatgtaactccttaggataatcaatatacaaaattccatgacaattggcgcccaacgtggggctcgaatataagtcgggtttatttgtaaattatccctagggacctccgagcatagcgggaggcatataaaagccaatagacaatggctagcaggaagtaatgttgaagaatatgaacttgatgttgaagctctggttgtaattttaagagatagaaatataccaagaaatcctttacatggagaagttataggtcttcgccttactgaaggatggtggggacaaattgagagatttcagatggtacgttgatctaaggctatggatttggccatgggacaagaaatattagtttatagtcccattgtatctatgactaaaatacaaaaaactccactaccagaaagaaaagctttacccattagatggataacatggatgacttatttagaagatccaagaatccaatttcattatgataaaaccttaccagaacttaagcatattccagatgtatatacatctagtcagtctcctgttaaacatccttctcaatatgaaggagtgttttatactgatggctcggccatcaaaagtcctgatcctacaaaaagcaataatgctggcatgggaatagtacatgccacatacaaacctgaatatcaagttttgaatcaatggtcaataccactaggtaatcatactgctcagatggctgaaatagctgcagttgaatttgcctgtaaaaaagctttaaaaatacctggtcctgtattagttataactgatagtttctatgtagcagaaagtgctaataaagaattaccatactggaaatctaatgggtttgttaataataagaaaaagcctcttaaacatatctccaaatggaaatctattgctgagtgtttatctatgaaaccagacattactattcaacatgaaaaaggcatcagcctacaaataccagtattcatactgaaaggcaatgccctagcagataagcttgccacccaaggaagttatgtggttaattgtaataccaaaaaaccaaacctggatgcagagttggatcaattattacagggtcattatataaaaggatatcccaaacaatatacatattttttagaagatggcaaagtaaaagtttccagacctgaaggggttaaaattattccccctcagtcagacagacaaaaaattgtgcttcaagcccacaatttggctcacaccggacgtgaagccactcttttaaaaattgccaacctttattggtggccaaatatgagaaaggatgtggttaaacaactaggacgctgtcaacagtgtttaatcacaaatgcttccaacaaagcctctggtcctattctaagaccagataggcctcaaaaaccttttgataaattctttattgactatattggacctttgccaccttcacagggatacctatatgtattagtagttgttgatggaatgacaggattcacttggttataccccactaaggctccttctactagcgcaactgttaaatctctcaatgtactcactagtattgcaattccaaaggtgattcactctgatcaaggtgcagcattcacttcttcaacctttgctgaatgggcaaaggaaagaggtatacatttggaattcagtactccttatcacccccaaagtggtagtaaggtggaaaggaaaaatagtgatataaaacgacttttaactaaactgctagtaggaagacccacaaagtggtatgacctattgcctgttgtacaacttgctttaaacaacacctatagccctgtattaaaatatactccacatcaactcttatttggtatagattcaaatactccatttgcaaatcaagatacacttgacttgaccagagaagaagaactttctcttttacaggaaattcgtacttctttataccatccatccacccctccagcctcctctcgttcctggtctcctgttgttggccaattggtccaggagagggtggctaggcctgcttctttgagacctcgttggcataaaccgtctactgtacttaaggtgttgaatccaaggactgttgttattttggaccatcttggcaacaacagaactgtaagtatagataatttaaaacctacttctcatcagaatggcaccaccaatgacactgcaacaatggatcatttggaaaaaaatgaataaagcgcatgaggcacttcaaaatacaacaactgtgactgaacagcagaaggaacaaattatactggacattcaaaatgaagaagtacaaccaactaggagagataaatttagatatctgctttatacttgttgtgctactagctcaagagtattggcctggatgtttttagtttgtatattgttaatcattgttttggtttcatgctttgtgactatatccagaatacaatggaataaggatattcaggtattaggacctgtaatagactggaatgttactcaaagagctgtttatcaacccttacagactagaaggattgcacgttcccttagaatgcagcatcctgttccaaaatatgtggaggtaaatatgactagtattccacaaggtgtatactatgaaccccatccggcctcgacggtatcgatggtaccggtatcgataagcttgataacctcgagagatctaattctaccgggtaggggaggcgcttttcccaaggcagtctggagcatgcgctttagcagccccgctggcacttggcgctacacaagtggcctctggcctcgcacacattccacatccaccggtagcgccaaccggctccgttctttggtggccccttcgcgccacttctactcctcccctagtcaggaagtttcccccagcaagctcgcgtcgtgcaggacgtgacaaatggaagtagcacgtctcactagtctcgtgcagatggacagcaccgctgagcaatggaagcgggtaggcctttggggcagcggccaatagcagctttgttccttcgctttctgggctcagaggctgggaaggggtgggtccgggggcgggctcaggggcgggctcaggggcgggcgggcgcccgaaggtcctcccgaggcccggcattctgcacgcttcaaaagcgcacgtctgccgcgctgttctcctcttcctcatctccgggcctttcgacctgcagcccgggggatcgatcctaggtgatttaaatccaccatgaccgagtacaagcccacggtgcgcctcgccacccgcgacgacgtcccccgggccgtacgcaccctcgccgccgcgttcgccgactaccccgccacgcgccacaccgtcgacccggaccgccacatcgagcgggtcaccgagctgcaagaactcttcctcacgcgcgtcgggctcgacatcggcaaggtgtgggtcgcggacgacggcgccgcggtggcggtctggaccacgccggagagcgtcgaagcgggggcggtgttcgccgagatcggcccgcgcatggccgagttgagcggttcccggctggccgcgcagcaacagatggaaggcctcctggcgccgcaccggcccaaggagcccgcgtggttcctggccaccgtcggcgtctcgcccgaccaccagggcaagggtctgggcagcgccgtcgtgctccccggagtggaggcggccgagcgcgccggggtgcccgccttcctggagacctccgcgccccgcaacctccccttctacgagcggctcggcttcaccgtcaccgccgacgtcgagtgcccgaaggaccgcgcgacctggtgcatgacccgcaagcccggtgcctgacggatccatcgctccggtgcccgtcagtgggcagagcgcacatcgcccacagtccccgagaagttggggggaggggtcggcaattgaaccggtgcctagagaaggtggcgcggggtaaactgggaaagtgatgtcgtgtactggctccgcctttttcccgagggtgggggagaaccgtatataagtgcagtagtcgccgtgaacgttctttttcgcaacgggtttgccgccagaacacagctgcggccgcgttaaccatgagccgatccgtggcactggctgtcctggctctgctgtctctgagtggcctggaagcagtgatggcccctagaacactgttcctgggcggaggcggctccggaggaggagggtctggaggcgggggaagtatccagcggactcccaagattcaggtctacagcagacaccctgccgaaaacgggaaatccaacttcctgaattgctatgtgtcaggctttcatcccagcgacatcgaggtcgatctgctgaagaatggcgagcggattgaaaaagtggagcactctgacctgtcattcagcaaggattggagcttttacctgctgtactatactgagtttaccccaacagaaaaagacgagtatgcctgtagggtgaaccatgtcaccctgagtcagcccaagatcgtgaaatgggaccgcgatatgggcgggggaggctccgggggaggcggctccggcggcgggggaagtggcgggggaggatccggttctcactccttgaagtatttccacacttccgtgtcccggcccggccgcggggagccccgcttcatctctgtgggctacgtggacgacacccagttcgtgcgcttcgacaacgacgccgcgagtccgaggatggtgccgcgggcgccgtggatggagcaggaggggtcagagtattgggaccgggagacacggagcgccagggacaccgcacagattttccgagtgaatctgcggacgctgcgcggctactacaatcagagcgaggccgggtctcacaccctgcagtggatgcatggctgcgagctggggcccgacgggcgcttcctccgcgggtatgaacagttcgcctacgacggcaaggattatctcaccctgaatgaggacctgcgctcctggaccgcggtggacacggcggctcagatctccgagcaaaagtcaaatgatgcctctgaggcggagcaccagagagcctacctggaagacacatgcgtggagtggctccacaaatacctggagaaggggaaggagacgctgcttcacctggagcccccaaagacacacgtgactcaccaccccatctctgaccatgaggccaccctgaggtgctgggccctgggcttctaccctgcggagatcacactgacctggcagcaggatggggagggccatacccaggacacggagctcgtggagaccaggcctgcaggggatggaaccttccagaagtgggcagctgtggtggtgccttctggagaggagcagagatacacgtgccatgtgcagcatgaggggctacccgagcccgtcaccctgagatggaagccggcttcccagcccaccatccccatcgtgggcatcattgctggcctggttctccttggatctgtggtctctggagctgtggttgctgctgtgatatggaggaagaagagctcaggtggaaaaggagggagctactctaaggctgagtggagcgacagtgcccaggggtctgagtctcacagcttgtaatctagagcggccgcgactctagatcaggcgcgccgttaccaagcagctatggaagcttatggacctcagagaggaagtaacgaggagagggtgtggtggaatgtcactagaaaccagggaaaacaaggaggagagtattacagggaaggaggtgaagaacctcattacccaaatactcctgctcctcatagacgtacctgggatgagagacacaaggttcttaaattgtcctcattcgctactccctctgacatccaacgctggactactaactctagattgtacgggaggctcttcactactcgctgcgtcgagagtgtacgagactctccaggtttggtaagaaatattttatattgttataatgttactatgatccattaacactctgcttatagattgtaagggtgattgcaatgctttctgcataaaactttggttttcttgttaatcaataaaccgacttgattcgagaaccaactcctatattattgtctcttttatactttattaagtaaaaggatttgtatattagccttgctaagggagacatctagtgatataagtgtgaactacacttatcttaaatgatgtaactccttaggataatcaatatacaaaattccatgacaattggcgataccgtcgaccgttcagctgcattaatgaatcggccaacgcgcggggagaggcggtttgcgtattgggcgctcttccgcttcctcgctcactgactcgctgcgctcggtcgttcggctgcggcgagcggtatcagctcactcaaaggcggtaatacggttatccacagaatcaggggataacgcaggaaagaacatgtgagcaaaaggccagcaaaaggccaggaaccgtaaaaaggccgcgttgctggcgtttttccataggctccgcccccctgacgagcatcacaaaaatcgacgctcaagtcagaggtggcgaaacccgacaggactataaagataccaggcgtttccccctggaagctccctcgtgcgctctcctgttccgaccctgccgcttaccggatacctgtccgcctttctcccttcgggaagcgtggcgctttctcaatgctcacgctgtaggtatctcagttcggtgtaggtcgttcgctccaagctgggctgtgtgcacgaaccccccgttcagcccgaccgctgcgccttatccggtaactatcgtcttgagtccaacccggtaagacacgacttatcgccactggcagcagccactggtaacaggattagcagagcgaggtatgtaggcggtgctacagagttcttgaagtggtggcctaactacggctacactagaaggacagtatttggtatctgcgctctgctgaagccagttaccttcggaaaaagagttggtagctcttgatccggcaaacaaaccaccgctggtagcggtggtttttttgtttgcaagcagcagattacgcgcagaaaaaaaggatctcaagaagatcctttgatcttttctacggggtctgacgctcagtggaacgaaaactcacgttaagggattttggtcatgagattatcaaaaaggatcttcacctagatccttttaaattaaaaatgaagttttaaatcaatctaaagtatatatgagtaaacttggtctgacagttaccaatgcttaatcagtgaggcacctatctcagcgatctgtctatttcgttcatccatagttgcctgactccccgtcgtgtagataactacgatacgggagggcttaccatctggccccagtgctgcaatgataccgcgagacccacgctcaccggctccagatttatcagcaataaaccagccagccggaagggccgagcgcagaagtggtcctgcaactttatccgcctccatccagtctattaattgttgccgggaagctagagtaagtagttcgccagttaatagtttgcgcaacgttgttgccattgctacaggcatcgtggtgtcacgctcgtcgtttggtatggcttcattcagctccggttcccaacgatcaaggcgagttacatgatcccccatgttgtgcaaaaaagcggttagctccttcggtcctccgatcgttgtcagaagtaagttggccgcagtgttatcactcatggttatggcagcactgcataattctcttactgtcatgccatccgtaagatgcttttctgtgactggtgagtactcaaccaagtcattctgagaatagtgtatgcggcgaccgagttgctcttgcccggcgtcaatacgggataataccgcgccacatagcagaactttaaaagtgctcatcattggaaaacgttcttcggggcgaaaactctcaaggatcttaccgctgttgagatccagttcgatgtaacccactcgtgcacccaactgatcttcagcatcttttactttcaccagcgtttctgggtgagcaaaaacaggaaggcaaaatgccgcaaaaaagggaataagggcgacacggaaatgttgaatactcatactcttcctttttcaatattattgaagcatttatcagggttattgtctcatgagcggatacatatttgaatgtatttagaaaaataaacaaataggggttccgcgcacatttccccgaaaagtgccacctgacgtctaagaaaccattattatcatgacattaacctataaaaataggcgtatcacgaggccctttcgtc

SEQ ID NO: 20 - protein, 500 aa, Artificial Sequence
  HLA-bGBE
MSRSVALAVLALLSLSGLEAVMAPRTLFLGGGGSGGGGSGGGGSIQRTPKIQVYSRHPAENGKSNFLNCYVSGFHPSDIEVDLLKNGERIEKVEHSDLSFSKDWSFYLLYYTEFTPTEKDEYACRVNHVTLSQPKIVKWDRDMGGGGSGGGGSGGGGSGGGGSGSHSLKYFHTSVSRPGRGEPRFISVGYVDDTQFVRFDNDAASPRMVPRAPWMEQEGSEYWDRETRSARDTAQIFRVNLRTLRGYYNQSEAGSHTLQWMHGCELGPDGRFLRGYEQFAYDGKDYLTLNEDLRSWTAVDTAAQISEQKSNDASEAEHQRAYLEDTCVEWLHKYLEKGKETLLHLEPPKTHVTHHPISDHEATLRCWALGFYPAEITLTWQQDGEGHTQDTELVETRPAGDGTFQKWAAVVVPSGEEQRYTCHVQHEGLPEPVTLRWKPASQPTIPIVGIIAGLVLLGSVVSGAVVAAVIWRKKSSGGKGGSYSKAEWSDSAQGSESHSL

SEQ ID NO: 21 - DNA, 7159 bp, Artificial Sequence
  Vector sequence for pA2-B2METKNpA
ctgcgcgctcgctcgctcactgaggccgcccgggcaaagcccgggcgtcgggcgacctttggtcgcccggcctcagtgagcgagcgagcgcgcagagagggagtggccaactccatcactaggggttcctgcggccgcgatgcagtccaaactctcactaaaattgccgagccctttgtcttccagtgtctaaaatattaatgtcaatggaatcaggccagagtttgaattctagtctcttagcctttgtttcccctgtccataaaatgaatgggggtaattctttcctcctacagtttatttatatattcactaattcattcattcatccatccattcgttcattcggtttactgagtacctactatgtgccagcccctgttctagggtggaaactaagagaatgatgtacctagagggcgctggaagctctaaagccctagcagttactgcttttactattagtggtcgtttttttctcccccccgccccccgacaaatcaacagaacaaagaaaattacctaaacagcaaggacatagggaggaacttcttggcacagaactttccaaacactttttcctgaagggatacaagaagcaagaaaggtactctttcactaggaccttctctgagctgtcctcaggatgcttttgggactatttttcttacccagagaatggagaaaccctgcagggaattcccaagctgtagttataaacagaagttctccttctgctaggtagcattcaaagatcttaatcttctgggtttccgttttctcgaatgaaaaatgcaggtccgagcagttaactggctggggcaccattagcaagtcacttagcatctctggggccagtctgcaaagcgagggggcagccttaatgtgcctccagcctgaagtcctagaatgagcgcccggtgtcccaagctggggcgcgcaccccagatcggagggcgccgatgtacagacagcaaactcacccagtctagtgcatgccttcttaaacatcacgagactctaagaaaaggaaactgaaaacgggaaagtccctctctctaacctggcactgcgtcgctggcttggagacaggtgacggtccctgcgggccttgtcctgattggctgggcacgcgtttaatataagtggaggcgtcgcgctggcgggcattcctgaagctgacagcattcgggccgagatctagataacttcgtataatgtatgctatacgaagttatggatccatcgattctgcgatcgctccggtgcccgtcagtgggcagagcgcacatcgcccacagtccccgagaagttggggggaggggtcggcaattgaaccggtgcctagagaaggtggcgcggggtaaactgggaaagtgatgtcgtgtactggctccgcctttttcccgagggtgggggagaaccgtatataagtgcagtagtcgccgtgaacgttctttttcgcaacgggtttgccgccagaacacagctgaagcttccaccatgcccacgctactgcgggtttatatagacggtccccacgggatggggaaaaccaccaccacgcaactgctggtggccctgggttcgcgcgacgatatcgtctacgtacccgagccgatgacttactggcgggtgctgggggcttccgagacaatcgcgaacatctacaccacacaacaccgcctcgaccagggtgagatatcggccggggacgcggcggtggtaatgacaagcgcccagataacaatgggcatgccttatgccgtgaccgacgccgttctggctcctcatatcgggggggaggctgggagctcacatgccccgcccccggccctcaccctcatcttcgaccgccatcccatcgccgccctcctgtgctacccggccgcgcggtaccttatgggcagcatgaccccccaggccgtgctggcgttcgtggccctcatcccgccgaccttgcccggcaccaacatcgtgcttggggcccttccggaggacagacacatcgaccgcctggccaaacgccagcgccccggcgagcggctggacctggctatgctggctgcgattcgccgcgtttacgggctacttgccaatacggtgcggtatctgcagtgcggcgggtcgtggcgggaggactggggacagctttcggggacggccgtgccgccccagggtgccgagccccagagcaacgcgggcccacgaccccatatcggggacacgttatttaccctgtttcgggcccccgagttgctggcccccaacggcgacctgtataacgtgtttgcctgggccttggacgtcttggccaaacgcctccgttccatgcacgtctttatcctggattacgaccaatcgcccgccggctgccgggacgccctgctgcaacttacctccgggatggtccagacccacgtcaccacccccggctccataccgacgatatgcgacctggcgcgcacgtttgcccgggagatgggatcggccattgaacaagatggattgcacgcaggttctccggccgcttgggtggagaggctattcggctatgactgggcacaacagacaatcggctgctctgatgccgccgtgttccggctgtcagcgcaggggcgcccggttctttttgtcaagaccgacctgtccggtgccctgaatgaactgcaggacgaggcagcgcggctatcgtggctggccacgacgggcgttccttgcgcagctgtgctcgacgttgtcactgaagcgggaagggactggctgctattgggcgaagtgccggggcaggatctcctgtcatctcaccttgctcctgccgagaaagtatccatcatggctgatgcaatgcggcggctgcatacgcttgatccggctacctgcccattcgaccaccaagcgaaacatcgcatcgagcgagcacgtactcggatggaagccggtcttgtcgatcaggatgatctggacgaagagcatcaggggctcgcgccagccgaactgttcgccaggctcaaggcgcgcatgcccgacggcgaggatctcgtcgtgacccatggcgatgcctgcttgccgaatatcatggtggaaaatggccgcttttctggattcatcgactgtggccggctgggtgtggcggaccgctatcaggacatagcgttggctacccgtgatattgctgaagagcttggcggcgaatgggctgaccgcttcctcgtgctttacggtatcgccgctcccgattcgcagcgcatcgccttctatcgccttcttgacgagttcttctgagggtctctagcataacttcgtataatgtatgctatacgaagttataataaaagatccttattttcattggatctgtgtgttggttttttgtgtgggatccgtcgataccgtcgactgtctcgctccgtggccttagctgtgctcgcgctactctctctttctggcctggaggctatccagcgtgagtctctcctaccctcccgctctggtccttcctctcccgctctgcaccctctgtggccctcgctgtgctctctcgctccgtgacttcccttctccaagttctccttggtggcccgccgtggggctagtccagggctggatctcggggaagcggcggggtggcctgggagtggggaagggggtgcgcacccgggacgcgcgctacttgcccctttcggcggggagcaggggagacctttggcctacggcgacgggagggtcgggacaaagtttagggcgtcgataagcgtcagagcgccgaggttgggggagggtttctcttccgctctttcgcggggcctctggctcccccagcgcagctggagtgggggacgggtaggctcgtcccaaaggcgcggcgctgaggtttgtgaacgcgtggaggggcgcttggggtctgggggaggcgtcgcccgggtaagcctgtctgctgcggctctgcttcccttagactggagagctgtggacttcgtctaggcgcccgctaagttcgcatgtcctagcacctctgggtctatgtggggccacaccgtggggaggaaacagcacgcgacgtttgtagaatgcttggctgtgatacaaagcggtttcgaataattaacttatttgttcccatcacatgtcacttttaaaaaattataagaactacccgttattgacatctttctgtgtgccaaggactttatgtgctttgcgtcatttaattttgaaaacagttatcttccgccatagataactactatggttatcttctgcctctcacagatgaagaaactaaggcaccgagattttaagaaacttaattacacaggggataaatggcagcaatcgagattgaagtcaagcctaaccagggcttttgcgggagcgcatgccttttggctgtaattcgtgcgcggccgcaggaacccctagtgatggagttggccactccctctctgcgcgctcgctcgctcactgaggccgggcgaccaaaggtcgcccgacgcccgggctttgcccgggcggcctcagtgagcgagcgagcgcgcagctgcctgcaggggcgcctgatgcggtattttctccttacgcatctgtgcggtatttcacaccgcatacgtcaaagcaaccatagtacgcgccctgtagcggcgcattaagcgcggcgggtgtggtggttacgcgcagcgtgaccgctacacttgccagcgccctagcgcccgctcctttcgctttcttcccttcctttctcgccacgttcgccggctttccccgtcaagctctaaatcgggggctccctttagggttccgatttagtgctttacggcacctcgaccccaaaaaacttgatttgggtgatggttcacgtagtgggccatcgccctgatagacggtttttcgccctttgacgttggagtccacgttctttaatagtggactcttgttccaaactggaacaacactcaaccctatctcgggctattcttttgatttataagggattttgccgatttcggcctattggttaaaaaatgagctgatttaacaaaaatttaacgcgaattttaacaaaatattaacgtttacaattttatggtgcactctcagtacaatctgctctgatgccgcatagttaagccagccccgacacccgccaacacccgctgacgcgccctgacgggcttgtctgctcccggcatccgcttacagacaagctgtgaccgtctccgggagctgcatgtgtcagaggttttcaccgtcatcaccgaaacgcgcgagacgaaagggcctcgtgatacgcctatttttataggttaatgtcatgataataatggtttcttagacgtcaggtggcacttttcggggaaatgtgcgcggaacccctatttgtttatttttctaaatacattcaaatatgtatccgctcatgagacaataaccctgataaatgcttcaataatattgaaaaaggaagagtatgagtattcaacatttccgtgtcgcccttattcccttttttgcggcattttgccttcctgtttttgctcacccagaaacgctggtgaaagtaaaagatgctgaagatcagttgggtgcacgagtgggttacatcgaactggatctcaacagcggtaagatccttgagagttttcgccccgaagaacgttttccaatgatgagcacttttaaagttctgctatgtggcgcggtattatcccgtattgacgccgggcaagagcaactcggtcgccgcatacactattctcagaatgacttggttgagtactcaccagtcacagaaaagcatcttacggatggcatgacagtaagagaattatgcagtgctgccataaccatgagtgataacactgcggccaacttacttctgacaacgatcggaggaccgaaggagctaaccgcttttttgcacaacatgggggatcatgtaactcgccttgatcgttgggaaccggagctgaatgaagccataccaaacgacgagcgtgacaccacgatgcctgtagcaatggcaacaacgttgcgcaaactattaactggcgaactacttactctagcttcccggcaacaattaatagactggatggaggcggataaagttgcaggaccacttctgcgctcggcccttccggctggctggtttattgctgataaatctggagccggtgagcgtgggtctcgcggtatcattgcagcactggggccagatggtaagccctcccgtatcgtagttatctacacgacggggagtcaggcaactatggatgaacgaaatagacagatcgctgagataggtgcctcactgattaagcattggtaactgtcagaccaagtttactcatatatactttagattgatttaaaacttcatttttaatttaaaaggatctaggtgaagatcctttttgataatctcatgaccaaaatcccttaacgtgagttttcgttccactgagcgtcagaccccgtagaaaagatcaaaggatcttcttgagatcctttttttctgcgcgtaatctgctgcttgcaaacaaaaaaaccaccgctaccagcggtggtttgtttgccggatcaagagctaccaactctttttccgaaggtaactggcttcagcagagcgcagataccaaatactgtccttctagtgtagccgtagttaggccaccacttcaagaactctgtagcaccgcctacatacctcgctctgctaatcctgttaccagtggctgctgccagtggcgataagtcgtgtcttaccgggttggactcaagacgatagttaccggataaggcgcagcggtcgggctgaacggggggttcgtgcacacagcccagcttggagcgaacgacctacaccgaactgagatacctacagcgtgagctatgagaaagcgccacgcttcccgaagggagaaaggcggacaggtatccggtaagcggcagggtcggaacaggagagcgcacgagggagcttccagggggaaacgcctggtatctttatagtcctgtcgggtttcgccacctctgacttgagcgtcgatttttgtgatgctcgtcaggggggcggagcctatggaaaaacgccagcaacgcggcctttttacggttcctggccttttgctggccttttgctcacatgtcctgcaggcag

SEQ ID NO: 22 - DNA, 7199 bp, Artificial Sequence
  Vector sequence for  pA2-B2MEHyTKpA
cctgcaggcagctgcgcgctcgctcgctcactgaggccgcccgggcaaagcccgggcgtcgggcgacctttggtcgcccggcctcagtgagcgagcgagcgcgcagagagggagtggccaactccatcactaggggttcctgcggccgcgaaactaagagaatgatgtacctagagggcgctggaagctctaaagccctagcagttactgcttttactattagtggtcgtttttttctcccccccgccccccgacaaatcaacagaacaaagaaaattacctaaacagcaaggacatagggaggaacttcttggcacagaactttccaaacactttttcctgaagggatacaagaagcaagaaaggtactctttcactaggaccttctctgagctgtcctcaggatgcttttgggactatttttcttacccagagaatggagaaaccctgcagggaattcccaagctgtagttataaacagaagttctccttctgctaggtagcattcaaagatcttaatcttctgggtttccgttttctcgaatgaaaaatgcaggtccgagcagttaactggctggggcaccattagcaagtcacttagcatctctggggccagtctgcaaagcgagggggcagccttaatgtgcctccagcctgaagtcctagaatgagcgcccggtgtcccaagctggggcgcgcaccccagatcggagggcgccgatgtacagacagcaaactcacccagtctagtgcatgccttcttaaacatcacgagactctaagaaaaggaaactgaaaacgggaaagtccctctctctaacctggcactgcgtcgctggcttggagacaggtgacggtccctgcgggccttgtcctgattggctgggcacgcgtttaatataagtggaggcgtcgcgctggcgggcattcctgaagctgacagcattcgggccgagatctagataacttcgtataatgtatgctatacgaagttatggatccatcgattctgcgatcgctccggtgcccgtcagtgggcagagcgcacatcgcccacagtccccgagaagttggggggaggggtcggcaattgaaccggtgcctagagaaggtggcgcggggtaaactgggaaagtgatgtcgtgtactggctccgcctttttcccgagggtgggggagaaccgtatataagtgcagtagtcgccgtgaacgttctttttcgcaacgggtttgccgccagaacacagctgaagcttccaccatgaaaaagcctgaactcaccgcgacgtctgtcgagaagtttctgatcgaaaagttcgacagcgtctccgacctgatgcagctctcggagggcgaagaatctcgtgctttcagcttcgatgtaggagggcgtggatatgtcctgcgggtaaatagctgcgccgatggtttctacaaagatcgttatgtttatcggcactttgcatcggccgcgctcccgattccggaagtgcttgacattggggaattcagcgagagcctgacctattgcatctcccgccgtgcacagggtgtcacgttgcaagacctgcctgaaaccgaactgcccgctgttctgcagccggtcgcggaggccatggatgcgatcgctgcggccgatcttagccagacgagcgggttcggcccattcggaccgcaaggaatcggtcaatacactacatggcgtgatttcatatgcgcgattgctgatccccatgtgtatcactggcaaactgtgatggacgacaccgtcagtgcgtccgtcgcgcaggctctcgatgagctgatgctttgggccgaggactgccccgaagtccggcacctcgtgcacgcggatttcggctccaacaatgtcctgacggacaatggccgcataacagcggtcattgactggagcgaggcgatgttcggggattcccaatacgaggtcgccaacatcttcttctggaggccgtggttggcttgtatggagcagcagacgcgctacttcgagcggaggcatccggagcttgcaggatcgccgcggctccgggcgtatatgctccgcattggtcttgaccaactctatcagagcttggttgacggcaatttcgatgatgcagcttgggcgcagggtcgatgcgacgcaatcgtccgatccggagccgggactgtcgggcgtacacaaatcgcccgcagaagcgcggccgtctggaccgatggctgtgtagaagtcgcgtctgcgttcgaccaggctgcgcgttctcgcggccatagcaaccgacgtacggcgttgcgccctcgccggcagcaagaagccacggaagtccgcccggagcagaaaatgcccacgctactgcgggtttatatagacggtccccacgggatggggaaaaccaccaccacgcaactgctggtggccctgggttcgcgcgacgatatcgtctacgtacccgagccgatgacttactggcgggtgctgggggcttccgagacaatcgcgaacatctacaccacacaacaccgcctcgaccagggtgagatatcggccggggacgcggcggtggtaatgacaagcgcccagataacaatgggcatgccttatgccgtgaccgacgccgttctggctcctcatatcgggggggaggctgggagctcacatgccccgcccccggccctcaccctcatcttcgaccgccatcccatcgccgccctcctgtgctacccggccgcgcggtaccttatgggcagcatgaccccccaggccgtgctggcgttcgtggccctcatcccgccgaccttgcccggcaccaacatcgtgcttggggcccttccggaggacagacacatcgaccgcctggccaaacgccagcgccccggcgagcggctggacctggctatgctggctgcgattcgccgcgtttacgggctacttgccaatacggtgcggtatctgcagtgcggcgggtcgtggcgggaggactggggacagctttcggggacggccgtgccgccccagggtgccgagccccagagcaacgcgggcccacgaccccatatcggggacacgttatttaccctgtttcgggcccccgagttgctggcccccaacggcgacctgtataacgtgtttgcctgggccttggacgtcttggccaaacgcctccgttccatgcacgtctttatcctggattacgaccaatcgcccgccggctgccgggacgccctgctgcaacttacctccgggatggtccagacccacgtcaccacccccggctccataccgacgatatgcgacctggcgcgcacgtttgcccgggagatgggggaggctaactgaggtctctagcataacttcgtataatgtatgctatacgaagttataataaaagatccttattttcattggatctgtgtgttggttttttgtgtgggatccgtcgataccgtcgactgtctcgctccgtggccttagctgtgctcgcgctactctctctttctggcctggaggctatccagcgtgagtctctcctaccctcccgctctggtccttcctctcccgctctgcaccctctgtggccctcgctgtgctctctcgctccgtgacttcccttctccaagttctccttggtggcccgccgtggggctagtccagggctggatctcggggaagcggcggggtggcctgggagtggggaagggggtgcgcacccgggacgcgcgctacttgcccctttcggcggggagcaggggagacctttggcctacggcgacgggagggtcgggacaaagtttagggcgtcgataagcgtcagagcgccgaggttgggggagggtttctcttccgctctttcgcggggcctctggctcccccagcgcagctggagtgggggacgggtaggctcgtcccaaaggcgcggcgctgaggtttgtgaacgcgtggaggggcgcttggggtctgggggaggcgtcgcccgggtaagcctgtctgctgcggctctgcttcccttagactggagagctgtggacttcgtctaggcgcccgctaagttcgcatgtcctagcacctctgggtctatgtggggccacaccgtggggaggaaacagcacgcgacgtttgtagaatgcttggctgtgatacaaagcggtttcgaataattaacttatttgttcccatcacatgtcacttttaaaaaattataagaactacccgttattgacatctttctgtgtgccaaggactttatgtgctttgcgtcatttaattttgaaaacagttatcttccgccatagataactactatggttatcttctgcctctcacagatgaagaaactaaggcaccgagattttaagaaacttaattacacaggggataaatggcagcaatcgagattgaagtcaagcctaaccagggcttttgcgggagcgcatgccttttggctgtaattcgtgcgcggccgcaggaacccctagtgatggagttggccactccctctctgcgcgctcgctcgctcactgaggccgggcgaccaaaggtcgcccgacgcccgggctttgcccgggcggcctcagtgagcgagcgagcgcgcagctgcctgcaggggcgcctgatgcggtattttctccttacgcatctgtgcggtatttcacaccgcatacgtcaaagcaaccatagtacgcgccctgtagcggcgcattaagcgcggcgggtgtggtggttacgcgcagcgtgaccgctacacttgccagcgccctagcgcccgctcctttcgctttcttcccttcctttctcgccacgttcgccggctttccccgtcaagctctaaatcgggggctccctttagggttccgatttagtgctttacggcacctcgaccccaaaaaacttgatttgggtgatggttcacgtagtgggccatcgccctgatagacggtttttcgccctttgacgttggagtccacgttctttaatagtggactcttgttccaaactggaacaacactcaaccctatctcgggctattcttttgatttataagggattttgccgatttcggcctattggttaaaaaatgagctgatttaacaaaaatttaacgcgaattttaacaaaatattaacgtttacaattttatggtgcactctcagtacaatctgctctgatgccgcatagttaagccagccccgacacccgccaacacccgctgacgcgccctgacgggcttgtctgctcccggcatccgcttacagacaagctgtgaccgtctccgggagctgcatgtgtcagaggttttcaccgtcatcaccgaaacgcgcgagacgaaagggcctcgtgatacgcctatttttataggttaatgtcatgataataatggtttcttagacgtcaggtggcacttttcggggaaatgtgcgcggaacccctatttgtttatttttctaaatacattcaaatatgtatccgctcatgagacaataaccctgataaatgcttcaataatattgaaaaaggaagagtatgagtattcaacatttccgtgtcgcccttattcccttttttgcggcattttgccttcctgtttttgctcacccagaaacgctggtgaaagtaaaagatgctgaagatcagttgggtgcacgagtgggttacatcgaactggatctcaacagcggtaagatccttgagagttttcgccccgaagaacgttttccaatgatgagcacttttaaagttctgctatgtggcgcggtattatcccgtattgacgccgggcaagagcaactcggtcgccgcatacactattctcagaatgacttggttgagtactcaccagtcacagaaaagcatcttacggatggcatgacagtaagagaattatgcagtgctgccataaccatgagtgataacactgcggccaacttacttctgacaacgatcggaggaccgaaggagctaaccgcttttttgcacaacatgggggatcatgtaactcgccttgatcgttgggaaccggagctgaatgaagccataccaaacgacgagcgtgacaccacgatgcctgtagcaatggcaacaacgttgcgcaaactattaactggcgaactacttactctagcttcccggcaacaattaatagactggatggaggcggataaagttgcaggaccacttctgcgctcggcccttccggctggctggtttattgctgataaatctggagccggtgagcgtgggtctcgcggtatcattgcagcactggggccagatggtaagccctcccgtatcgtagttatctacacgacggggagtcaggcaactatggatgaacgaaatagacagatcgctgagataggtgcctcactgattaagcattggtaactgtcagaccaagtttactcatatatactttagattgatttaaaacttcatttttaatttaaaaggatctaggtgaagatcctttttgataatctcatgaccaaaatcccttaacgtgagttttcgttccactgagcgtcagaccccgtagaaaagatcaaaggatcttcttgagatcctttttttctgcgcgtaatctgctgcttgcaaacaaaaaaaccaccgctaccagcggtggtttgtttgccggatcaagagctaccaactctttttccgaaggtaactggcttcagcagagcgcagataccaaatactgtccttctagtgtagccgtagttaggccaccacttcaagaactctgtagcaccgcctacatacctcgctctgctaatcctgttaccagtggctgctgccagtggcgataagtcgtgtcttaccgggttggactcaagacgatagttaccggataaggcgcagcggtcgggctgaacggggggttcgtgcacacagcccagcttggagcgaacgacctacaccgaactgagatacctacagcgtgagctatgagaaagcgccacgcttcccgaagggagaaaggcggacaggtatccggtaagcggcagggtcggaacaggagagcgcacgagggagcttccagggggaaacgcctggtatctttatagtcctgtcgggtttcgccacctctgacttgagcgtcgatttttgtgatgctcgtcaggggggcggagcctatggaaaaacgccagcaacgcggcctttttacggttcctggccttttgctggccttttgctcacatgt

SEQ ID NO: 23 - protein, 29 aa, Artificial Sequence
  HLA-G peptide
MAPRTLFLGGGGSGGGGSGGGGSIQRTPK

SEQ ID NO: 24 - DNA, 1369 bp, Homo sapiens
  CDS (506)..(1219)
ccggacgccgcacggctcctgttccggtgtcagagggcccgccctccccgctcctcagtctttgcggacaagaaaggggctgtgtgagacgcagggaaggaggcacacccgggggtggcgcagtgaggagggggcgcgacggccaggaggctggtggagcgacacccaggcaggagagggggaagaactctctccctttctgaacccccttttccttgagagacgagttgggggagtcctccacgcattacccactcgggccgcaaaaactcccttctttagccctctgcccccgcccttgcttataagcctttgagaccgcagaagggaccttgttgtggaacgggacggccaagaggaagccagatcgctgagggtccggtctccagtttgcctcctgctatatccattggaagagaaaagtttgtgacttgggcccccaagttttgagagaactgggctttcggcgcggggggacagaggaggctcgtggggagctttccccatggagcttacccagcctgcagaagacctcatccagacccagcagacccctgcctcagaacttggggaccctgaagaccccggagaggaggctgcagatggctcagacactgtggtcctcagtctctttccctgcacccctgagcctgtgaatcctgaaccggatgccagtgtttcctctccacagggcagctccctgaagcactccaccactctcaccaaccggcagcgagggaacgaggtgtcagctctgccggccaccctagactgtgacaacctcgtcaacaagccagacgagcgcggcttcacccccctcatctgggcctccgcctttggagagattgagaccgttcgcttcctgctggagtggggtgccgacccccacatcctggcaaaagagcgagagagcgccctgtcgctggccagcacaggcggctacacagacattgtggggctgctgctggagcgtgacgtggacatcaacatctatgattggaatggagggacgccactgctgtacgctgtgcgcgggaaccacgtgaaatgcgttgaggccttgctggcccgaggcgctgacctcaccaccgaagccgactctggctacaccccgatggaccttgccgtggccctgggataccggaaagtgcaacaggtgatcgagaaccacatcctcaagctcttccagagcaacctggtgcccgctgaccctgagtgaaggccgcctgccggggactcagacactcagggaacaaaatggtcagccagagctggggaaacccagaactgacttcaaaggcagcttctggacaggtggtgggaggggacccttcccaagaggaaccaataaaccttctgtgcagaatga

SEQ ID NO: 25 - protein, 237 aa, Homo sapiens
MELTQPAEDLIQTQQTPASELGDPEDPGEEAADGSDTVVLSLFPCTPEPVNPEPDASVSSPQGSSLKHSTTLTNRQRGNEVSALPATLDCDNLVNKPDERGFTPLIWASAFGEIETVRFLLEWGADPHILAKERESALSLASTGGYTDIVGLLLERDVDINIYDWNGGTPLLYAVRGNHVKCVEALLARGADLTTEADSGYTPMDLAVALGYRKVQQVIENHILKLFQSNLVPADPE

SEQ ID NO: 26 - DNA, 1438 bp, Homo sapiens
  CDS (506)..(1288)
ccggacgccgcacggctcctgttccggtgtcagagggcccgccctccccgctcctcagtctttgcggacaagaaaggggctgtgtgagacgcagggaaggaggcacacccgggggtggcgcagtgaggagggggcgcgacggccaggaggctggtggagcgacacccaggcaggagagggggaagaactctctccctttctgaacccccttttccttgagagacgagttgggggagtcctccacgcattacccactcgggccgcaaaaactcccttctttagccctctgcccccgcccttgcttataagcctttgagaccgcagaagggaccttgttgtggaacgggacggccaagaggaagccagatcgctgagggtccggtctccagtttgcctcctgctatatccattggaagagaaaagtttgtgacttgggcccccaagttttgagagaactgggctttcggcgcggggggacagaggaggctcgtggggagctttccccatggagcttacccagcctgcagaagacctcatccagacccagcagacccctgcctcagaacttggggaccctgaagaccccggagaggaggctgcagatggctcagacactgtggtcctcagtctctttccctgcacccctgagcctgtgaatcctgaaccggatgccagtgtttcctctccacaggcaggcagctccctgaagcactccaccactctcaccaaccggcagcgagggaacgaggtgtcagctctgccggccaccctagactccctgtccatccaccagctcgcagcacagggggagctggaccagctgaaggagcatttgcggaaaggtgacaacctcgtcaacaagccagacgagcgcggcttcacccccctcatctgggcctccgcctttggagagattgagaccgttcgcttcctgctggagtggggtgccgacccccacatcctggcaaaagagcgagagagcgccctgtcgctggccagcacaggcggctacacagacattgtggggctgctgctggagcgtgacgtggacatcaacatctatgattggaatggagggacgccactgctgtacgctgtgcgcgggaaccacgtgaaatgcgttgaggccttgctggcccgaggcgctgacctcaccaccgaagccgactctggctacaccccgatggaccttgccgtggccctgggataccggaaagtgcaacaggtgatcgagaaccacatcctcaagctcttccagagcaacctggtgcccgctgaccctgagtgaaggccgcctgccggggactcagacactcagggaacaaaatggtcagccagagctggggaaacccagaactgacttcaaaggcagcttctggacaggtggtgggaggggacccttcccaagaggaaccaataaaccttctgtgcagaatga

SEQ ID NO: 27 - protein, 260 aa, Homo sapiens
MELTQPAEDLIQTQQTPASELGDPEDPGEEAADGSDTVVLSLFPCTPEPVNPEPDASVSSPQAGSSLKHSTTLTNRQRGNEVSALPATLDSLSIHQLAAQGELDQLKEHLRKGDNLVNKPDERGFTPLIWASAFGEIETVRFLLEWGADPHILAKERESALSLASTGGYTDIVGLLLERDVDINIYDWNGGTPLLYAVRGNHVKCVEALLARGADLTTEADSGYTPMDLAVALGYRKVQQVIENHILKLFQSNLVPADPE

SEQ ID NO: 28 - DNA, 3618 bp, Homo sapiens
  CDS (222)..(2072)
attcagaaaaaggaaaataaagcaacgcacgagccggctgggccaggaccttggggctgggctggagtgaaggtggctacgagttttccagatttaggagacttcagaaaggtggggcagatagaatggagatggcaaagatctctttgggcatatatgggcctggcgaagtaatggaataatttctaattttcggagaaggcaagtgccctcatgccgggatggcagaagatgagcctgatgctaagagccccaagactgggggaagggcccccccaggtggtgctgaggctggggaacctaccacccttcttcagaggctccgaggtaccatttccaaggccgtgcagaacaaagtagaggggatcctgcaagatgtacagaaattttctgacaatgacaagctgtatctctaccttcagctcccctcaggacccaccactggagacaaaagctcagagccaagtacactgagcaatgaggagtacatgtatgcctataggtggatccgcaaccacctggaagagcacactgacacctgtctgccaaagcaaagtgtttatgatgcctatcggaagtactgtgagagtcttgcctgttgccgcccactcagcacagccaactttggcaagatcatcagagagatcttccctgacatcaaagctcgaaggcttggtggccggggccagtccaaatattgctacagtggcataaggaggaagaccttggtgtctatgccacccctgcctggacttgacctaaagggttctgagagtccagaaatgggcccagaagtaaccccagcacctcgagatgaactggtggaggcagcgtgtgccctgacctgtgactgggcagagcggatcctgaaacggtccttcagttccatcgttgaggtcgcccgcttcctgctacagcagcatctcatctctgcccgatctgcacatgcccatgtgcttaaggccatggggcttgctgaagaggacgaacatgcacctcgggaacggtcatctaaaccaaagaatggtttagagaacccagagggtggagcccacaagaagccagagagactggcccagcctcctaaggatctggaagcccgaactggggccggtcctctcgcacgtggagagcggaagaagagtgtagttgagagctcggccccaggagccaataacctgcaggttaatgccctagtggctcggctgcctctgctccttccccgggcccctcgctcactaattccgccaatcccagtctctccacctattctggcccccaggctttcttcaggtgccctgaaagtggctacactgcctctgtctagtagggccggggcacccccagcagctgtgcccatcattaacatgatcttaccaactgttcctgctttgcctggacctggacctgggcctgggcgagctccacctgggggactcactcagccccggggcacagagaacagagaggtaggcataggtggtgaccaaggaccacatgacaagggtgtcaagaggacagctgaagtacctgtgagtgaggccagtgggcaggctccaccagctaaagcagcaaagcaggatatagaggatacagcaagtgatgccaaaaggaaacgggggcgccctcgaaaaaagtcaggtggaagtggggaaaggaattctacccctctcaagtcagcagctgccatggaatctgcccagtcctcaaggttaccatgggagacatggggctcaggaggggaaggcaactcagctggaggggcagagaggccagggccaatgggagaggctgaaaagggggcagtacttgcccagggtcagggagatggtactgtttccaaaggaggaaggggccccggttcccagcataccaaagaagcagaagataaaattcccttggtcccctcaaaagtgagtgtcatcaagggcagcagaagccaaaaggaggcttttcctttggcaaagggagaggtagacactgcaccacagggtaataaagacttaaaggagcatgtgcttcaaagttccttatcccaggagcataaagacccaaaagcaacacccccatgatacaggtctgtggggaagagtgtttatatccctacgttaactttgcctagtagaggcccttctttgcacttgcttctcatttggctattcttttcctaaggaagtccattctcctctgtacagacagctgagtcacccagtctacttagtacctggttgctgcctctgaccttttcagcttgataccctgggctttagtgtaaccaataaatctgtagtgaccttacctgtattccctgtgctatcctgtgggaaggtaggaatgggctaagtatgatgaatatataggttagggatcttttggttttaaatcacagaaaacctaattcaaactggcttaaaataaaaaggatttattggttcatgtaactagaaagtccataggtagtgctggctccaggtgaagacttgacccagtagttcagtatgtctctaaataccggactgacttttttctcactgttgcatcttctgtaggaccatttaagtctgggccacttaatggctgccagcattcctaagattacacttttccccatttatgtccaatcagaaaaagaaggcatctttgtaccagaaatctcagcaaaagccctaatattcacactgattaggcctgggtcacatgtccaccctgaccaatcactgtggccaggaggatgatacatgctaatttgcttattctatatcatggacaacacctttggggaaaagggtgggggtcagcctccccaaaatcacatggattccccaagtggaaactaggagcagggagttgcttgggtggccgctaacaccaggctactcttattttagcttgctaagttgagatcagctagacctgctttcttttctcctcagtcttgcatttccctcaatacaagctgtagcctctttcctcgtttctagtctcagaaggaaggagagggaagccattctcctctagggactcttcagtctcatttagatgatagtccctttttttctacctccatattagagatggagctccttccttttcctgtttcttaatttttgtcttctcattcctgcttccctctcaccctattgccagttccaccaactagagtgaaagacttcctagccatttcattaaatctattctgtatccaccaggtggcagcatcttgtcatacgtgtcaggacttaggactgcggggtttaggttagatgtcacggaaaaagctagttctgtggtcaggcggcaccaatgagaaaggaatgcagaccctccagatgtatccttgggaaaagcagtaaaccaactaatatttattgaagacctactttgtcctctacatagggtagcttctgtcagggaatcttggttcttcccaagaaacactgattttctttcagggagacttcatgtgttcatttatttccaccacagcagattttaagaaattataatatgtaatatttgatatctataaagagtatatctaacgtgaataaattatgaagcatactaatgagtacctatgacccataacacatatacattaaaacattttaaatacca

SEQ ID NO: 29 - protein, 616 aa, Homo sapiens
MAEDEPDAKSPKTGGRAPPGGAEAGEPTTLLQRLRGTISKAVQNKVEGILQDVQKFSDNDKLYLYLQLPSGPTTGDKSSEPSTLSNEEYMYAYRWIRNHLEEHTDTCLPKQSVYDAYRKYCESLACCRPLSTANFGKIIREIFPDIKARRLGGRGQSKYCYSGIRRKTLVSMPPLPGLDLKGSESPEMGPEVTPAPRDELVEAACALTCDWAERILKRSFSSIVEVARFLLQQHLISARSAHAHVLKAMGLAEEDEHAPRERSSKPKNGLENPEGGAHKKPERLAQPPKDLEARTGAGPLARGERKKSVVESSAPGANNLQVNALVARLPLLLPRAPRSLIPPIPVSPPILAPRLSSGALKVATLPLSSRAGAPPAAVPIINMILPTVPALPGPGPGPGRAPPGGLTQPRGTENREVGIGGDQGPHDKGVKRTAEVPVSEASGQAPPAKAAKQDIEDTASDAKRKRGRPRKKSGGSGERNSTPLKSAAAMESAQSSRLPWETWGSGGEGNSAGGAERPGPMGEAEKGAVLAQGQGDGTVSKGGRGPGSQHTKEAEDKIPLVPSKVSVIKGSRSQKEAFPLAKGEVDTAPQGNKDLKEHVLQSSLSQEHKDPKATPP

SEQ ID NO: 30 - DNA, 3611 bp, Homo sapiens
  CDS (215)..(2065)
attcagaaaaaggaaaataaagcaacgcacgagccggctgggccaggaccttggggctgggctggagtgaaggtggctacgagttttccagatttaggagacttcagaaaggtggggcagatagaatggagatggcaaagatctctttgggcatatatgggcctggcgaagtaatggaataatttctaattttcggagaagccctcatgccgggatggcagaagatgagcctgatgctaagagccccaagactgggggaagggcccccccaggtggtgctgaggctggggaacctaccacccttcttcagaggctccgaggtaccatttccaaggccgtgcagaacaaagtagaggggatcctgcaagatgtacagaaattttctgacaatgacaagctgtatctctaccttcagctcccctcaggacccaccactggagacaaaagctcagagccaagtacactgagcaatgaggagtacatgtatgcctataggtggatccgcaaccacctggaagagcacactgacacctgtctgccaaagcaaagtgtttatgatgcctatcggaagtactgtgagagtcttgcctgttgccgcccactcagcacagccaactttggcaagatcatcagagagatcttccctgacatcaaagctcgaaggcttggtggccggggccagtccaaatattgctacagtggcataaggaggaagaccttggtgtctatgccacccctgcctggacttgacctaaagggttctgagagtccagaaatgggcccagaagtaaccccagcacctcgagatgaactggtggaggcagcgtgtgccctgacctgtgactgggcagagcggatcctgaaacggtccttcagttccatcgttgaggtcgcccgcttcctgctacagcagcatctcatctctgcccgatctgcacatgcccatgtgcttaaggccatggggcttgctgaagaggacgaacatgcacctcgggaacggtcatctaaaccaaagaatggtttagagaacccagagggtggagcccacaagaagccagagagactggcccagcctcctaaggatctggaagcccgaactggggccggtcctctcgcacgtggagagcggaagaagagtgtagttgagagctcggccccaggagccaataacctgcaggttaatgccctagtggctcggctgcctctgctccttccccgggcccctcgctcactaattccgccaatcccagtctctccacctattctggcccccaggctttcttcaggtgccctgaaagtggctacactgcctctgtctagtagggccggggcacccccagcagctgtgcccatcattaacatgatcttaccaactgttcctgctttgcctggacctggacctgggcctgggcgagctccacctgggggactcactcagccccggggcacagagaacagagaggtaggcataggtggtgaccaaggaccacatgacaagggtgtcaagaggacagctgaagtacctgtgagtgaggccagtgggcaggctccaccagctaaagcagcaaagcaggatatagaggatacagcaagtgatgccaaaaggaaacgggggcgccctcgaaaaaagtcaggtggaagtggggaaaggaattctacccctctcaagtcagcagctgccatggaatctgcccagtcctcaaggttaccatgggagacatggggctcaggaggggaaggcaactcagctggaggggcagagaggccagggccaatgggagaggctgaaaagggggcagtacttgcccagggtcagggagatggtactgtttccaaaggaggaaggggccccggttcccagcataccaaagaagcagaagataaaattcccttggtcccctcaaaagtgagtgtcatcaagggcagcagaagccaaaaggaggcttttcctttggcaaagggagaggtagacactgcaccacagggtaataaagacttaaaggagcatgtgcttcaaagttccttatcccaggagcataaagacccaaaagcaacacccccatgatacaggtctgtggggaagagtgtttatatccctacgttaactttgcctagtagaggcccttctttgcacttgcttctcatttggctattcttttcctaaggaagtccattctcctctgtacagacagctgagtcacccagtctacttagtacctggttgctgcctctgaccttttcagcttgataccctgggctttagtgtaaccaataaatctgtagtgaccttacctgtattccctgtgctatcctgtgggaaggtaggaatgggctaagtatgatgaatatataggttagggatcttttggttttaaatcacagaaaacctaattcaaactggcttaaaataaaaaggatttattggttcatgtaactagaaagtccataggtagtgctggctccaggtgaagacttgacccagtagttcagtatgtctctaaataccggactgacttttttctcactgttgcatcttctgtaggaccatttaagtctgggccacttaatggctgccagcattcctaagattacacttttccccatttatgtccaatcagaaaaagaaggcatctttgtaccagaaatctcagcaaaagccctaatattcacactgattaggcctgggtcacatgtccaccctgaccaatcactgtggccaggaggatgatacatgctaatttgcttattctatatcatggacaacacctttggggaaaagggtgggggtcagcctccccaaaatcacatggattccccaagtggaaactaggagcagggagttgcttgggtggccgctaacaccaggctactcttattttagcttgctaagttgagatcagctagacctgctttcttttctcctcagtcttgcatttccctcaatacaagctgtagcctctttcctcgtttctagtctcagaaggaaggagagggaagccattctcctctagggactcttcagtctcatttagatgatagtccctttttttctacctccatattagagatggagctccttccttttcctgtttcttaatttttgtcttctcattcctgcttccctctcaccctattgccagttccaccaactagagtgaaagacttcctagccatttcattaaatctattctgtatccaccaggtggcagcatcttgtcatacgtgtcaggacttaggactgcggggtttaggttagatgtcacggaaaaagctagttctgtggtcaggcggcaccaatgagaaaggaatgcagaccctccagatgtatccttgggaaaagcagtaaaccaactaatatttattgaagacctactttgtcctctacatagggtagcttctgtcagggaatcttggttcttcccaagaaacactgattttctttcagggagacttcatgtgttcatttatttccaccacagcagattttaagaaattataatatgtaatatttgatatctataaagagtatatctaacgtgaataaattatgaagcatactaatgagtacctatgacccataacacatatacattaaaacattttaaatacca

SEQ ID NO: 31 - protein, 616 aa, Homo sapiens; identical to SEQ ID NO: 29

SEQ ID NO: 32 - DNA, 2825 bp, Homo sapiens
  CDS (157)..(975)
cgcgcaggctgcggtcgcgcaggcgcagtcggggcgccttcccggtataggcgccttttaccccagcgtgtcctgagtctttggttcgcgaagtgccgttaggccaagcaggtgctaaaagcccggggtcgtggaccccggccaggtcttagcagcatggaggcgcagggtgtagcggagggcgcggggccgggcgccgccagcggcgtgccccaccccgcggccctagccccggctgcggctcccaccttggcgccagcctcggtggcggccgcggcctctcaattcaccctgctagtgatgcaaccctgtgctgggcaggacgaggctgcggcccccgggggcagcgttggggcgggcaagcccgttaggtacctgtgcgaaggggccggggatggcgaagaggaggctggggaggacgaggcggacctgttagacacttcggaccctccggggggaggcgagagcgcggctagtttggaggatctagaggacgaggagactcactcggggggcgagggcagcagcgggggcgcccggaggcggggcagcggtgggggcagcatgagcaagacctgcacctacgaaggctgcagcgagaccacgagccaggtggccaagcagcgcaaaccgtggatgtgcaagaaacaccgcaacaagatgtacaaggacaagtataaaaagaagaagagcgaccaggccctgaactgcggtgggactgcctcgactggcagcgcgggaaacgtcaaactcgaggaaagtgcagataacatactctccattgttaaacaaagaacaggatcttttggggatcgtcctgcaagacctactcttttagaacaagtgttaaatcaaaaaagactgtcgttactaagaagtccagaagtagtgcaatttttacagaaacagcaacagctattaaatcagcaagttttggagcaaagacaacagcagtttccaggaacatcaatgtgagggaacttaccaagaacatctacatggttttttatcttattgtaatagatgagcatatttttttaccagacataaatggggtaataatctatgcctgtagaacataaacattttcctgtaaatgtatgtgtgcatttggggataagtaagtattgcactttgtgcatctaatctttcagattactgtgagtttgaagaagtcagcttatctttccaaataacatttaattataatgttttttaaaaaatatattcctcttcagtcattgttactgaaggtaatgaagcagttactttctgtggaagtcataaagttaatagatattaatcttgactcatctagctcagtggttctcatcaagggtcaatttgattgtcatagtgaccttgaaaaccactggcttttagtgagtggccaggaatgctaaatgttctgcagtgtcaggggtagtcccacatactaaagattgtctcacccgcagtgccaataacactcctaagaaatgttgatggctattttgtggtgctaacatgtagttggggcacctataattgggttctcttaataacctttctttgcagttaagactgaagctgtcaaagaggtaagcacattttatatagacgtaaggaaagtgattattgtttaatatctgtgaatttaggatgtgcatctcttttcagaggtgtgttagtaaaacctgacggattaactaagcacactgggatgtgtctcctacagttggcttctctctttgatgttacctgttagtgctgatctcttaaagcagacatttcttgtttgttgaatttgtgaacagtatagatctcagcccaccaatgccaagacaaaattatttttcttatacttattttttattaaacaaaatgaaaaagatccttttcaaaaaggtgatcctgaaaataaaactaacactccagtattttgtcattgtttttcgcaattgagctatctgaaaactgttattcctaagtaatgttcaaaaatgataagtaatctggatacctttttcttatactttctcctaggaaaactttaaaactttaaaaaggcaaacctaccaataggaataacaaattaaatgtcaagagagtatatccaatattaggatataaatgtatgtgtctcaagtttaactctacaaaaatttgttacttgttttttaaactctatatataaagttcgacttaatcatggctgttctaagaagtacttatggagagcaagaacgtttttgttcatttcttaatgtgtgtgtttttacttgcatatctgttcaaaacacttttaacaaaattaattcattaaagtccagttgttgacctttgagttagctgatttctttattctgttctttagtttattcttactagatgcagaggaattcatctactgtctgttattaactgttagtttattctcatacttacgatgttgagagtttttttgaagcttaagttaccctttatggtggaaaacattagcttatgcttctttagatggaataatgggaaaggagggaaatgggaaatggatggaaatgggaaaggagggaaaataatagcccagtgagagctgaatgaaaagggactgaatttaaatatttgtaagaactttgtgatgatgagtaattgtcagacgtgggatagataactgagaggctcagaatctttaccaaggatattttttaggataaggtagctgcctgttcatgaatttggataagaatagtaggacaatattcaacacaatttaatttttgtctgccacattagacatttttttaccttataaaatgatcaataaagcaataaggtttattttgggt

SEQ ID NO: 33 - protein, 272 aa, Homo sapiens
MEAQGVAEGAGPGAASGVPHPAALAPAAAPTLAPASVAAAASQFTLLVMQPCAGQDEAAAPGGSVGAGKPVRYLCEGAGDGEEEAGEDEADLLDTSDPPGGGESAASLEDLEDEETHSGGEGSSGGARRRGSGGGSMSKTCTYEGCSETTSQVAKQRKPWMCKKHRNKMYKDKYKKKKSDQALNCGGTASTGSAGNVKLEESADNILSIVKQRTGSFGDRPARPTLLEQVLNQKRLSLLRSPEVVQFLQKQQQLLNQQVLEQRQQQFPGTSM

SEQ ID NO: 34 - DNA, 4654 bp, Homo sapiens
  CDS (134)..(3526)
ggttagtgatgaggctagtgatgaggctgtgtgcttctgagctgggcatccgaaggcatccttggggaagctgagggcacgaggaggggctgccagactccgggagctgctgcctggctgggattcctacacaatgcgttgcctggctccacgccctgctgggtcctacctgtcagagccccaaggcagctcacagtgtgccaccatggagttggggcccctagaaggtggctacctggagcttcttaacagcgatgctgaccccctgtgcctctaccacttctatgaccagatggacctggctggagaagaagagattgagctctactcagaacccgacacagacaccatcaactgcgaccagttcagcaggctgttgtgtgacatggaaggtgatgaagagaccagggaggcttatgccaatatcgcggaactggaccagtatgtcttccaggactcccagctggagggcctgagcaaggacattttcaagcacataggaccagatgaagtgatcggtgagagtatggagatgccagcagaagttgggcagaaaagtcagaaaagacccttcccagaggagcttccggcagacctgaagcactggaagccagctgagccccccactgtggtgactggcagtctcctagtgggaccagtgagcgactgctccaccctgccctgcctgccactgcctgcgctgttcaaccaggagccagcctccggccagatgcgcctggagaaaaccgaccagattcccatgcctttctccagttcctcgttgagctgcctgaatctccctgagggacccatccagtttgtccccaccatctccactctgccccatgggctctggcaaatctctgaggctggaacaggggtctccagtatattcatctaccatggtgaggtgccccaggccagccaagtaccccctcccagtggattcactgtccacggcctcccaacatctccagaccggccaggctccaccagccccttcgctccatcagccactgacctgcccagcatgcctgaacctgccctgacctcccgagcaaacatgacagagcacaagacgtcccccacccaatgcccggcagctggagaggtctccaacaagcttccaaaatggcctgagccggtggagcagttctaccgctcactgcaggacacgtatggtgccgagcccgcaggcccggatggcatcctagtggaggtggatctggtgcaggccaggctggagaggagcagcagcaagagcctggagcgggaactggccaccccggactgggcagaacggcagctggcccaaggaggcctggctgaggtgctgttggctgccaaggagcaccggcggccgcgtgagacacgagtgattgctgtgctgggcaaagctggtcagggcaagagctattgggctggggcagtgagccgggcctgggcttgtggccggcttccccagtacgactttgtcttctctgtcccctgccattgcttgaaccgtccgggggatgcctatggcctgcaggatctgctcttctccctgggcccacagccactcgtggcggccgatgaggttttcagccacatcttgaagagacctgaccgcgttctgctcatcctagacggcttcgaggagctggaagcgcaagatggcttcctgcacagcacgtgcggaccggcaccggcggagccctgctccctccgggggctgctggccggccttttccagaagaagctgctccgaggttgcaccctcctcctcacagcccggccccggggccgcctggtccagagcctgagcaaggccgacgccctatttgagctgtccggcttctccatggagcaggcccaggcatacgtgatgcgctactttgagagctcagggatgacagagcaccaagacagagccctgacgctcctccgggaccggccacttcttctcagtcacagccacagccctactttgtgccgggcagtgtgccagctctcagaggccctgctggagcttggggaggacgccaagctgccctccacgctcacgggactctatgtcggcctgctgggccgtgcagccctcgacagcccccccggggccctggcagagctggccaagctggcctgggagctgggccgcagacatcaaagtaccctacaggaggaccagttcccatccgcagacgtgaggacctgggcgatggccaaaggcttagtccaacacccaccgcgggccgcagagtccgagctggccttccccagcttcctcctgcaatgcttcctgggggccctgtggctggctctgagtggcgaaatcaaggacaaggagctcccgcagtacctagcattgaccccaaggaagaagaggccctatgacaactggctggagggcgtgccacgctttctggctgggctgatcttccagcctcccgcccgctgcctgggagccctactcgggccatcggcggctgcctcggtggacaggaagcagaaggtgcttgcgaggtacctgaagcggctgcagccggggacactgcgggcgcggcagctgctggagctgctgcactgcgcccacgaggccgaggaggctggaatttggcagcacgtggtacaggagctccccggccgcctctcttttctgggcacccgcctcacgcctcctgatgcacatgtactgggcaaggccttggaggcggcgggccaagacttctccctggacctccgcagcactggcatttgcccctctggattggggagcctcgtgggactcagctgtgtcacccgtttcagggctgccttgagcgacacggtggcgctgtgggagtccctgcagcagcatggggagaccaagctacttcaggcagcagaggagaagttcaccatcgagcctttcaaagccaagtccctgaaggatgtggaagacctgggaaagcttgtgcagactcagaggacgagaagttcctcggaagacacagctggggagctccctgctgttcgggacctaaagaaactggagtttgcgctgggccctgtctcaggcccccaggctttccccaaactggtgcggatcctcacggccttttcctccctgcagcatctggacctggatgcgctgagtgagaacaagatcggggacgagggtgtctcgcagctctcagccaccttcccccagctgaagtccttggaaaccctcaatctgtcccagaacaacatcactgacctgggtgcctacaaactcgccgaggccctgccttcgctcgctgcatccctgctcaggctaagcttgtacaataactgcatctgcgacgtgggagccgagagcttggctcgtgtgcttccggacatggtgtccctccgggtgatggacgtccagtacaacaagttcacggctgccggggcccagcagctcgctgccagccttcggaggtgtcctcatgtggagacgctggcgatgtggacgcccaccatcccattcagtgtccaggaacacctgcaacaacaggattcacggatcagcctgagatgatcccagctgtgctctggacaggcatgttctctgaggacactaaccacgctggaccttgaactgggtacttgtggacacagctcttctccaggctgtatcccatgagcctcagcatcctggcacccggcccctgctggttcagggttggcccctgcccggctgcggaatgaaccacatcttgctctgctgacagacacaggcccggctccaggctcctttagcgcccagttgggtggatgcctggtggcagctgcggtccacccaggagccccgaggccttctctgaaggacattgcggacagccacggccaggccagagggagtgacagaggcagccccattctgcctgcccaggcccctgccaccctggggagaaagtacttctttttttttatttttagacagagtctcactgttgcccaggctggcgtgcagtggtgcgatctgggttcactgcaacctccgcctcttgggttcaagcgattcttctgcttcagcctcccgagtagctgggactacaggcacccaccatcatgtctggctaatttttcatttttagtagagacagggttttgccatgttggccaggctggtctcaaactcttgacctcaggtgatccacccacctcagcctcccaaagtgctgggattacaagcgtgagccactgcaccgggccacagagaaagtacttctccaccctgctctccgaccagacaccttgacagggcacaccgggcactcagaagacactgatgggcaacccccagcctgctaattccccagattgcaacaggctgggcttcagtggcagctgcttttgtctatgggactcaatgcactgacattgttggccaaagccaaagctaggcctggccagatgcaccagcccttagcagggaaacagctaatgggacactaatggggcggtgagaggggaacagactggaagcacagcttcatttcctgtgtcttttttcactacattataaatgtctctttaatgtcacaggcaggtccagggtttgagttcataccctgttaccattttggggtacccactgctctggttatctaatatgtaacaagccaccccaaatcatagtggcttaaaacaacactcacattta

SEQ ID NO: 35 - protein, 1130 aa, Homo sapiens
MRCLAPRPAGSYLSEPQGSSQCATMELGPLEGGYLELLNSDADPLCLYHFYDQMDLAGEEEIELYSEPDTDTINCDQFSRLLCDMEGDEETREAYANIAELDQYVFQDSQLEGLSKDIFKHIGPDEVIGESMEMPAEVGQKSQKRPFPEELPADLKHWKPAEPPTVVTGSLLVGPVSDCSTLPCLPLPALFNQEPASGQMRLEKTDQIPMPFSSSSLSCLNLPEGPIQFVPTISTLPHGLWQISEAGTGVSSIFIYHGEVPQASQVPPPSGFTVHGLPTSPDRPGSTSPFAPSATDLPSMPEPALTSRANMTEHKTSPTQCPAAGEVSNKLPKWPEPVEQFYRSLQDTYGAEPAGPDGILVEVDLVQARLERSSSKSLERELATPDWAERQLAQGGLAEVLLAAKEHRRPRETRVIAVLGKAGQGKSYWAGAVSRAWACGRLPQYDFVFSVPCHCLNRPGDAYGLQDLLFSLGPQPLVAADEVFSHILKRPDRVLLILDGFEELEAQDGFLHSTCGPAPAEPCSLRGLLAGLFQKKLLRGCTLLLTARPRGRLVQSLSKADALFELSGFSMEQAQAYVMRYFESSGMTEHQDRALTLLRDRPLLLSHSHSPTLCRAVCQLSEALLELGEDAKLPSTLTGLYVGLLGRAALDSPPGALAELAKLAWELGRRHQSTLQEDQFPSADVRTWAMAKGLVQHPPRAAESELAFPSFLLQCFLGALWLALSGEIKDKELPQYLALTPRKKRPYDNWLEGVPRFLAGLIFQPPARCLGALLGPSAAASVDRKQKVLARYLKRLQPGTLRARQLLELLHCAHEAEEAGIWQHVVQELPGRLSFLGTRLTPPDAHVLGKALEAAGQDFSLDLRSTGICPSGLGSLVGLSCVTRFRAALSDTVALWESLQQHGETKLLQAAEEKFTIEPFKAKSLKDVEDLGKLVQTQRTRSSSEDTAGELPAVRDLKKLEFALGPVSGPQAFPKLVRILTAFSSLQHLDLDALSENKIGDEGVSQLSATFPQLKSLETLNLSQNNITDLGAYKLAEALPSLAASLLRLSLYNNCICDVGAESLARVLPDMVSLRVMDVQYNKFTAAGAQQLAASLRRCPHVETLAMWTPTIPFSVQEHLQQQDSRISLR

SEQ ID NO: 36 - DNA, 1697 bp, Homo sapiens
  CDS (108)..(890)
atttccagtgctagaggcccacagtttcagtctcatctgcctccactcggcctcagttcctcatcactgttcctgtgctcacagtcatcaattatagaccccacaacatgcgccctgaagacagaatgttccatatcagagctgtgatcttgagagccctctccttggctttcctgctgagtctccgaggagctggggccatcaaggcggaccatgtgtcaacttatgccgcgtttgtacagacgcatagaccaacaggggagtttatgtttgaatttgatgaagatgagatgttctatgtggatctggacaagaaggagaccgtctggcatctggaggagtttggccaagccttttcctttgaggctcagggcgggctggctaacattgctatattgaacaacaacttgaataccttgatccagcgttccaaccacactcaggccaccaacgatccccctgaggtgaccgtgtttcccaaggagcctgtggagctgggccagcccaacaccctcatctgccacattgacaagttcttcccaccagtgctcaacgtcacgtggctgtgcaacggggagctggtcactgagggtgtcgctgagagcctcttcctgcccagaacagattacagcttccacaagttccattacctgacctttgtgccctcagcagaggacttctatgactgcagggtggagcactggggcttggaccagccgctcctcaagcactgggaggcccaagagccaatccagatgcctgagacaacggagactgtgctctgtgccctgggcctggtgctgggcctagtcggcatcatcgtgggcaccgtcctcatcataaagtctctgcgttctggccatgacccccgggcccaggggaccctgtgaaatactgtaaaggtgacaaaatatctgaacagaagaggacttaggagagatctgaactccagctgccctacaaactccatctcagcttttcttctcacttcatgtgaaaactactccagtggctgactgaattgctgacccttcaagctctgtccttatccattacctcaaagcagtcattccttagtaaagtttccaacaaatagaaattaatgacactttggtagcactaatatggagattatcctttcattgagccttttatcctctgttctcctttgaagaacccctcactgtcaccttcccgagaataccctaagaccaataaatacttcagtatttcagagcggggagactctgagtcattcttactggaagtctaggaccaggtcacatgtgaatactatttcttgaaggtgtggtttcaacctctgttgccgatgtggttactaaaggttctgatcccacttgaacggaaaggtctgaggatattgattcagtcctgggtttttccctaactacaggatagggtggggtagagaaaggatatttgggggaaattttacttggatgaagattttcttggatgtagtttgaagactgcagtgtttgaagtctctgagggaagagatttggtctgtctggatcaagatttcaggcagattaggattccattcacagcccctgagcttccttcccaaggctgtattgtaattatagcaatatttcatggaggatttttctacatgataaactaagagccaagaaataaaatttttaaaatgccctaaaaaaaaaaaaaaaaaa

SEQ ID NO: 37 - protein, 260 aa, Homo sapiens
MRPEDRMFHIRAVILRALSLAFLLSLRGAGAIKADHVSTYAAFVQTHRPTGEFMFEFDEDEMFYVDLDKKETVWHLEEFGQAFSFEAQGGLANIAILNNNLNTLIQRSNHTQATNDPPEVTVFPKEPVELGQPNTLICHIDKFFPPVLNVTWLCNGELVTEGVAESLFLPRTDYSFHKFHYLTFVPSAEDFYDCRVEHWGLDQPLLKHWEAQEPIQMPETTETVLCALGLVLGLVGIIVGTVLIIKSLRSGHDPRAQGTL

SEQ ID NO: 38 - DNA, 777 bp, Homo sapiens
  CDS (1)..(777)
atgatggttctgcaggtttctgcggccccccggacagtggctctgacggcgttactgatggtgctgctcacatctgtggtccagggcagggccactccagagaattacgtgtaccagggacggcaggaatgctacgcgtttaatgggacacagcgcttcctggagagatacatctacaaccgggaggagtacgcgcgcttcgacagcgacgtgggggagttccgggcggtgacggagctggggcggcctgctgcggagtactggaacagccagaaggacatcctggaggagaagcgggcagtgccggacagggtatgcagacacaactacgagctggacgaggccgtgaccctgcagcgccgagtccagcctaaggtgaacgtttccccctccaagaaggggcccctgcagcaccacaacctgcttgtctgccacgtgacagatttctacccaggcagcattcaagtccgatggttcctgaatggacaggaggaaacagctggggtcgtgtccaccaacctgatccgtaatggagactggaccttccagatcctggtgatgctggaaatgaccccccagcagggagacgtctacatctgccaagtggagcacaccagcctggacagtcctgtcaccgtggagtggaaggcacagtctgattctgcccagagtaagacattgacgggagctgggggcttcgtgctggggctcatcatctgtggagtgggcatcttcatgcacaggaggagcaagaaagttcaacgaggatctgcataa

SEQ ID NO: 39 - protein, 258 aa, Homo sapiens [sequence omitted]

SEQ ID NO: 40 - DNA, 768 bp, Homo sapiens
  CDS (1)..(768)
atgatcctaaacaaagctctgctgctgggggccctcgctctgaccaccgtgatgagcccctgtggaggtgaagacattgtggctgaccacgttgcctcttgtggtgtaaacttgtaccagttttacggtccctctggccagtacacccatgaatttgatggagatgaggagttctacgtggacctggagaggaaggagactgcctggcggtggcctgagttcagcaaatttggaggttttgacccgcagggtgcactgagaaacatggctgtggcaaaacacaacttgaacatcatgattaaacgctacaactctaccgctgctaccaatgaggttcctgaggtcacagtgttttccaagtctcccgtgacactgggtcagcccaacaccctcatttgtcttgtggacaacatctttcctcctgtggtcaacatcacatggctgagcaatgggcagtcagtcacagaaggtgtttctgagaccagcttcctctccaagagtgatcattccttcttcaagatcagttacctcaccttcctcccttctgctgatgagatttatgactgcaaggtggagcactggggcctggaccagcctcttctgaaacactgggagcctgagattccagcccctatgtcagagctcacagagactgtggtctgcgccctggggttgtctgtgggcctcgtgggcattgtggtgggcactgtcttcatcatccaaggcctgcgttcagttggtgcttccagacaccaagggccattgtga

SEQ ID NO: 41 - protein, 255 aa, Homo sapiens [sequence omitted]

SEQ ID NO: 42 - DNA, 786 bp, Homo sapiens
  CDS (1)..(786)
atgtcttggaaaaaggctttgcggatccccggaggccttcgggcagcaactgtgaccttgatgctgtcgatgctgagcaccccagtggctgagggcagagactctcccgaggatttcgtgtaccagtttaagggcatgtgctacttcaccaacgggacagagcgcgtgcgtcttgtgagcagaagcatctataaccgagaagagatcgtgcgcttcgacagcgacgtgggggagttccgggcggtgacgctgctggggctgcctgccgccgagtactggaacagccagaaggacatcctggagaggaaacgggcggcggtggacagggtgtgcagacacaactaccagttggagctccgcacgaccttgcagcggcgagtggagcccacagtgaccatctccccatccaggacagaggccctcaaccaccacaacctgctggtctgctcggtgacagatttctatccagcccagatcaaagtccggtggtttcggaatgaccaggaggagacagctggcgttgtgtccaccccccttattaggaatggtgactggaccttccagatcctggtgatgctggaaatgactccccagcgtggagacgtctacacctgccacgtggagcaccccagcctccagagccccatcaccgtggagtggcgggctcaatctgaatctgcccagagcaagatgctgagtggcattggaggcttcgtgctggggctgatcttcctcgggctgggccttatcatccatcacaggagtcagaaagggctcctgcactga

SEQ ID NO: 43 - protein, 261 aa, Homo sapiens
MSWKKALRIPGGLRAATVTLMLSMLSTPVAEGRDSPEDFVYQFKGMCYFTNGTERVRLVSRSIYNREEIVRFDSDVGEFRAVTLLGLPAAEYWNSQKDILERKRAAVDRVCRHNYQLELRTTLQRRVEPTVTISPSRTEALNHHNLLVCSVTDFYPAQIKVRWFRNDQEETAGVVSTPLIRNGDWTFQILVMLEMTPQRGDVYTCHVEHPSLQSPITVEWRAQSESAQSKMLSGIGGFVLGLIFLGLGLIIHHRSQKGLLH

SEQ ID NO: 44 - DNA, 1312 bp, Homo sapiens
  CDS (110)..(874)
ttttaatggtcagactctattacaccccacattctcttttcttttattcttgtctgttctgcctcactcccgagctctactgactcccaacagagcgcccaagaagaaaatggccataagtggagtccctgtgctaggatttttcatcatagctgtgctgatgagcgctcaggaatcatgggctatcaaagaagaacatgtgatcatccaggccgagttctatctgaatcctgaccaatcaggcgagtttatgtttgactttgatggtgatgagattttccatgtggatatggcaaagaaggagacggtctggcggcttgaagaatttggacgatttgccagctttgaggctcaaggtgcattggccaacatagctgtggacaaagccaacctggaaatcatgacaaagcgctccaactatactccgatcaccaatgtacctccagaggtaactgtgctcacaaacagccctgtggaactgagagagcccaacgtcctcatctgtttcatagacaagttcaccccaccagtggtcaatgtcacgtggcttcgaaatggaaaacctgtcaccacaggagtgtcagagacagtcttcctgcccagggaagaccaccttttccgcaagttccactatctccccttcctgccctcaactgaggacgtttacgactgcagggtggagcactggggcttggatgagcctcttctcaagcactgggagtttgatgctccaagccctctcccagagactacagagaacgtggtgtgtgccctgggcctgactgtgggtctggtgggcatcattattgggaccatcttcatcatcaagggattgcgcaaaagcaatgcagcagaacgcagggggcctctgtaaggcacatggaggtgatggtgtttcttagagagaagatcactgaagaaacttctgctttaatggctttacaaagctggcaatattacaatccttgacctcagtgaaagcagtcatcttcagcattttccagccctatagccaccccaagtgtggatatgcctcttcgattgctccgtactctaacatctagctggcttccctgtctattgccttttcctgtatctattttcctctatttcctatcattttattatcaccatgcaatgcctctggaataaaacatacaggagtctgtctctgctatggaatgccccatggggcatctcttgtgtacttattgtttaaggtttcctcaaactgtgatttttctgaacacaataaactattttgatgatcttgggtggaaaaaaaaaaaaaaaaaaaaaaaaaaaaaaaaaa

SEQ ID NO: 45 - protein, 254 aa, Homo sapiens
MAISGVPVLGFFIIAVLMSAQESWAIKEEHVIIQAEFYLNPDQSGEFMFDFDGDEIFHVDMAKKETVWRLEEFGRFASFEAQGALANIAVDKANLEIMTKRSNYTPITNVPPEVTVLTNSPVELREPNVLICFIDKFTPPVVNVTWLRNGKPVTTGVSETVFLPREDHLFRKFHYLPFLPSTEDVYDCRVEHWGLDEPLLKHWEFDAPSPLPETTENVVCALGLTVGLVGIIIGTIFIIKGLRKSNAAERRGPL

SEQ ID NO: 46 - DNA, 801 bp, Homo sapiens
  CDS (1)..(801)
atggtgtgtctgaagctccctggaggctcctgcatgacagcgctgacagtgacactgatggtgctgagctccccactggctttggctggggacacccgaccacgtttcttgtggcagcttaagtttgaatgtcatttcttcaatgggacggagcgggtgcggttgctggaaagatgcatctataaccaagaggagtccgtgcgcttcgacagcgacgtgggggagtaccgggcggtgacggagctggggcggcctgatgccgagtactggaacagccagaaggacctcctggagcagaggcgggccgcggtggacacctactgcagacacaactacggggttggtgagagcttcacagtgcagcggcgagttgagcctaaggtgactgtgtatccttcaaagacccagcccctgcagcaccacaacctcctggtctgctctgtgagtggtttctatccaggcagcattgaagtcaggtggttccggaacggccaggaagagaaggctggggtggtgtccacaggcctgatccagaatggagattggaccttccagaccctggtgatgctggaaacagttcctcggagtggagaggtttacacctgccaagtggagcacccaagtgtgacgagccctctcacagtggaatggagagcacggtctgaatctgcacagagcaagatgctgagtggagtcgggggcttcgtgctgggcctgctcttccttggggccgggctgttcatctacttcaggaatcagaaaggacactctggacttcagccaacaggattcctgagctga

SEQ ID NO: 47 - protein, 266 aa, Homo sapiens
MVCLKLPGGSCMTALTVTLMVLSSPLALAGDTRPRFLWQLKFECHFFNGTERVRLLERCIYNQEESVRFDSDVGEYRAVTELGRPDAEYWNSQKDLLEQRRAAVDTYCRHNYGVGESFTVQRRVEPKVTVYPSKTQPLQHHNLLVCSVSGFYPGSIEVRWFRNGQEEKAGVVSTGLIQNGDWTFQTLVMLETVPRSGEVYTCQVEHPSVTSPLTVEWRARSESAQSKMLSGVGGFVLGLLFLGAGLFIYFRNQKGHSGLQPTGFLS

SEQ ID NO: 48 - DNA, 1122 bp, Homo sapiens
  CDS (87)..(872)
gatctaaggccaccctctcggggagggagttggggaagctgggttggctgggttggtagctcctacctactgtgtggcaagaaggtatgggtcatgaacagaaccaaggagctgcgctgctacagatgttaccacttctgtggctgctaccccactcctgggccgtccctgaagctcctactccaatgtggccagatgacctgcaaaaccacacattcctgcacacagtgtactgccaggatgggagtcccagtgtgggactctctgaggcctacgacgaggaccagcttttcttcttcgacttttcccagaacactcgggtgcctcgcctgcccgaatttgctgactgggctcaggaacagggagatgctcctgccattttatttgacaaagagttctgcgagtggatgatccagcaaatagggccaaaacttgatgggaaaatcccggtgtccagagggtttcctatcgctgaagtgttcacgctgaagcccctggagtttggcaagcccaacactttggtctgttttgtcagtaatctcttcccacccatgctgacagtgaactggcagcatcattccgtccctgtggaaggatttgggcctacttttgtctcagctgtcgatggactcagcttccaggccttttcttacttaaacttcacaccagaaccttctgacattttctcctgcattgtgactcacgaaattgaccgctacacagcaattgcctattgggtaccccggaacgcactgccctcagatctgctggagaatgtgctgtgtggcgtggcctttggcctgggtgtgctgggcatcatcgtgggcattgttctcatcatctacttccggaagccttgctcaggtgactgattcttccagaccagagtttgatgccagcagcttcggccatccaaacagaggatgctcagatttctcacatcctgcccaggatctcctcttagggtagaagtctctgggacatccctggggtgtgtgtgtagatttcccacctggggactctgctgtccctgggcttgcatcccagggatcccagagtggcctgcctatcacaaccacatcccttccccccacaaggcaataaatctcatttctttatatc

SEQ ID NO: 49 - protein, 261 aa, Homo sapiens
MGHEQNQGAALLQMLPLLWLLPHSWAVPEAPTPMWPDDLQNHTFLHTVYCQDGSPSVGLSEAYDEDQLFFFDFSQNTRVPRLPEFADWAQEQGDAPAILFDKEFCEWMIQQIGPKLDGKIPVSRGFPIAEVFTLKPLEFGKPNTLVCFVSNLFPPMLTVNWQHHSVPVEGFGPTFVSAVDGLSFQAFSYLNFTPEPSDIFSCIVTHEIDRYTAIAYWVPRNALPSDLLENVLCGVAFGLGVLGIIVGIVLIIYFRKPCSGD

SEQ ID NO: 50 - DNA, 1412 bp, Homo sapiens
  CDS (264)..(1055)
atttgtccctgcctacctagccaatctgtccctgtttgggacactggactcccgtgagctggaaggaacagatttaatatctaggggctgggtatccccacatcactcatttggggggtcaagggacccgggcaatatagtattctgctcagtgtctggagatcatctacccaggctggggcttctgggacaggcgaggacccacggaccctggaagagctggtccaggggactgaactcccggcatctttacagagcagagcatgatcacattcctgccgctgctgctggggctcagcctgggctgcacaggagcaggtggcttcgtggcccatgtggaaagcacctgtctgttggatgatgctgggactccaaaggatttcacatactgcatctccttcaacaaggatctgctgacctgctgggatccagaggagaataagatggccccttgcgaatttggggtgctgaatagcttggcgaatgtcctctcacagcacctcaaccaaaaagacaccctgatgcagcgcttgcgcaatgggcttcagaattgtgccacacacacccagcccttctggggatcactgaccaacaggacacggccaccatctgtgcaagtagccaaaaccactccttttaacacgagggagcctgtgatgctggcctgctatgtgtggggcttctatccagcagaagtgactatcacgtggaggaagaacgggaagcttgtcatgcctcacagcagtgcgcacaagactgcccagcccaatggagactggacataccagaccctctcccatttagccttaaccccctcttacggggacacttacacctgtgtggtagagcacactggggctcctgagcccatccttcgggactggacacctgggctgtcccccatgcagaccctgaaggtttctgtgtctgcagtgactctgggcctgggcctcatcatcttctctcttggtgtgatcagctggcggagagctggccactctagttacactcctcttcctgggtccaattattcagaaggatggcacatttcctagaggcagaatcctacaacttccactccaagtgagaaggagattcaaactcaatgatgctaccatgcctctccaacatcttcaaccccctgacattatcttggatcctatggtttctccatccaattctttgaatttcccagtctcccctatgtaaaacttagcaacttgggggacctcattcctgggactatgctgtaaccaaattattgtccaaggctatatttctgggatgaatataatctgaggaagggagttaaagaccctcctggggctctcagtgtgccatagaggacagcaactggtgattgtttcagagaaataaactttggtggaaatattgttaaaaaaaaaaaaaaa

SEQ ID NO: 51 - protein, 263 aa, Homo sapiens
MITFLPLLLGLSLGCTGAGGFVAHVESTCLLDDAGTPKDFTYCISFNKDLLTCWDPEENKMAPCEFGVLNSLANVLSQHLNQKDTLMQRLRNGLQNCATHTQPFWGSLTNRTRPPSVQVAKTTPFNTREPVMLACYVWGFYPAEVTITWRKNGKLVMPHSSAHKTAQPNGDWTYQTLSHLALTPSYGDTYTCVVEHTGAPEPILRDWTPGLSPMQTLKVSVSAVTLGLGLIIFSLGVISWRRAGHSSYTPLPGSNYSEGWHIS

SEQ ID NO: 52 - DNA, 3485 bp, Homo sapiens
  CDS (77)..(829)
cttcttctttacctccgccttgttcctgtcctcaccacacggactgagactgatttgattaaagcaccagagtgtaatggccctcagagcagggctggtcctggggttccacaccctgatgaccctcctgagcccgcaggaggcaggggccaccaaggctgaccacatgggctcctacggacccgccttctaccagtcttacggcgcctcgggccagttcacccatgaatttgatgaggaacagctgttctctgtggacctgaagaaaagcgaggccgtgtggcgtctgcctgagtttggtgactttgcccgctttgacccgcagggcgggctggccggcatcgccgcaatcaaagcccatctggacatcctggtggagcgctccaaccgcagcagagccatcaacgtgcctccacgggtgaccgtgctccccaagtctcgggtggagctgggccagcccaacatcctcatctgcatcgtggacaacatcttcccccctgtgatcaatatcacctggctgcgcaacggccaaactgtcactgagggagtggcccagaccagcttctattcccagcctgaccatttgttccgcaagttccactacctgcccttcgtgccctcagccgaggacgtctatgactgccaggtggagcactggggcctggatgcgccactcctcaggcattgggagctccaggtgcctattccaccaccagatgccatggagaccctggtctgtgccctgggcctggccatcggcctggtgggcttcctcgtgggcaccgtcctcatcatcatgggcacatatgtgtccagtgtccccaggtaatgatccttctgagagaaatgacttgtgggagacaccctgcagatcctcatgggtttgtgacagcccctgcgtgctcagtgccctttaagtgcatcccgctgtgctgactttgagtgggatcaacatctgtcctacgggtcccctcttttttggccccagtattcatggcagggtttgttggacacctactagcttcccttcccattcaacacacacacacattcttgctctacccaaagctctggctggcagcactaaatgctttggtggtgtttgcactgtgtcctttccaggccttggccagttcttccaggggtgaggcatgtggtgctggggattggcagccatcctggggcccacacaggtgtgtcttgctccatttggcccattgtgtgttactttgtgaatgagccatttcacatggacttcatgaaatttgcctcctgagttcaggtttaccctgaaagggatgcagattatcctgttcctcacgaccccctcagctaacaacagttctgaagggtgctgggacaggacaggctcatggggactccactcctgcctgggtttactctgtatgaagaggccactggtatcctgccatgatgttatctcctttttctacttttccctagagtcccatgcatgataaagagaggcccaaggcttggataaggtggccacttccctcagtggagtcagtcatgttaggtaggaggtggtagagtcggtctgcgaggtatctcgtaagaggggaggtccacctagacacactctaaatatgtggcctagaagattttggtctacttttctgtgaacagaatttaaaacatacaaagagataaatcaccataccacatagtttatgtcaggaccaaaatgagcaatacagattacggttttcaaaccagaatgcacataagaactgcttgggatccttttaaaagtacaggcattggcctggtgcagtggctcattcctgtaatcccagcactttgggaggccaaggggacaggactgcttgaggccaagaggtggaaaccatcttgggctacatagagagaccccatctctacaaagaaagatttaaaaattaaccaggcatggtggctcgcacctgtattcccagccactggggaggctgaggccggaggagtgcttgagcccaggagttcaaggctgcagtgagccaagattgcgccactgcactccagcctaggtgacagagtgagaccctgtctctaaataaataaataaataaaatataaaaataacagtcatcacccagacctactgaattagaatctcgggagtgcagggggcagcaacagggaggctgtcttttctgagatggggtctcactctgtcaccaggctggagtgccatggcatgatctcagctcactgcaacctccacctcctgagttcaagccattctcctgcctcagcctcctgagtagctgggactacaggtgtgcgccactacactcagctaatttttgtattttaagtagagacggggtttcatcatgttggccaggatggcctccatctcttgacctcgtgatccacccaccttccctcccaaagtactggaattacaggcattagccactgtgcccagccgaggctgtcatttttaaccggctctggatgactctgatgcagccatcctggaccttggctgtggtctggtaactggaacccagtgacgtaatcaggtgccatcgggggtcatgggaaagggggatccccaaggtctgaggtggactaggaaggctttctgaagaacctgggtctgttagggcatcagccaatcaaggtacaagtaaatagaggcaaaatgagggtttgaactgtgagcagttggtcctggaaaagaaagaaaccaagagattatggggactcaatgggcttcttaagagagaataagttgaaatcaatgaccagaagaccctgatggaagtggaggagaatcatctcaggcaaactttttgtgtgccagtaacagaaaccctctttgtgtgatcacatgcaaagtataggatatttgcaatatagccatggggaggagtgcagggcccaagggtagattttagccaggcctcccaggaacagaactcggatccgaaaagcccagagaagctagagctgcccctccaacactctcggatccacatggtctgtgttctctagacccccctgcatgttagcggtgttctctctctgtggactgactgtccttctcagtgaacatgtccacccgacagctcctgagtttatatcatctcaaccctcacaacccacagaggctgtgtctcctagtcacagctttaaattactggaaaaataaatgactggccaaacttggagcaggtgtccatcccagccctgtgtagttagagcaggaatcaagatctcaacacaaatgtggctgccaagcactcagccccggggcgaggggtcaagttcttctcagagaaagaggaataagttggttctcagaagacatcacaagatacgtgtgtacccaacaatctctgatctctgctgatcttttgcttagacgttaacttgatgcatcattggaaaggtgtttctctcatctctgtcctaaggcttgataaagtcattaaaattgtgttcttttgactaaa

SEQ ID NO: 53 - protein, 250 aa, Homo sapiens
MALRAGLVLGFHTLMTLLSPQEAGATKADHMGSYGPAFYQSYGASGQFTHEFDEEQLFSVDLKKSEAVWRLPEFGDFARFDPQGGLAGIAAIKAHLDILVERSNRSRAINVPPRVTVLPKSRVELGQPNILICIVDNIFPPVINITWLRNGQTVTEGVAQTSFYSQPDHLFRKFHYLPFVPSAEDVYDCQVEHWGLDAPLLRHWELQVPIPPPDAMETLVCALGLAIGLVGFLVGTVLIIMGTYVSSVPR

SEQ ID NO: 54 - DNA, 1388 bp, Homo sapiens
  CDS (98)..(919)
gatttatactcttaatgggtactttctgactgaattttatgagctcattctgaagaggctgacgattttactatctcatttttttcctttctccagaatgggttctgggtgggtcccctgggtggtggctctgctagtgaatctgacccgactggattcctccatgactcaaggcacagactctccagaagattttgtgattcaggcaaaggctgactgttacttcaccaacgggacagaaaaggtgcagtttgtggtcagattcatctttaacttggaggagtatgtacgtttcgacagtgatgtggggatgtttgtggcattgaccaagctggggcagccagatgctgagcagtggaacagccggctggatctcttggagaggagcagacaggccgtggatggggtctgtagacacaactacaggctgggcgcacccttcactgtggggagaaaagtgcaaccagaggtgacagtgtacccagagaggaccccactcctgcaccagcataatctgctgcactgctctgtgacaggcttctatccaggggatatcaagatcaagtggttcctgaatgggcaggaggagagagctggggtcatgtccactggccctatcaggaatggagactggacctttcagactgtggtgatgctagaaatgactcctgaacttggacatgtctacacctgccttgtcgatcactccagcctgctgagccctgtttctgtggagtggagagctcagtctgaatattcttggagaaagatgctgagtggcattgcagccttcctacttgggctaatcttccttctggtgggaatcgtcatccagctaagggctcagaaaggatatgtgaggacgcagatgtctggtaatgaggtctcaagagctgttctgctccctcagtcatgctaaggtcctcactgaagcttctctctctggagcctgaagtagtgatgagtagtctgggccctgggtgaggtaaaggacattcatgaggtcaatgttctgggaataactctcttccctgatccttggaggagcccgaactgattctggagctctgtgttctgagatcatgcatctcccacccatctgcccttctcccttctacgtgtacatcattaatccccattgccaagggcattgtccagaaactcccctgagaccttactccttccagccccaaatcatttacttttctgtggtccagccctactcctataagtcatgatctccaaagctttctgtcttccaactgcagtctccacagtcttcagaagacaaatgctcaggtagtcactgtttccttttcactgtttttaaaaaccttttattgtcaaataaaatggagatacaaaaaatgtaaaaaaaaaaaaaaaaa

SEQ ID NO: 55 - protein, 273 aa, Homo sapiens
MGSGWVPWVVALLVNLTRLDSSMTQGTDSPEDFVIQAKADCYFTNGTEKVQFVVRFIFNLEEYVRFDSDVGMFVALTKLGQPDAEQWNSRLDLLERSRQAVDGVCRHNYRLGAPFTVGRKVQPEVTVYPERTPLLHQHNLLHCSVTGFYPGDIKIKWFLNGQEERAGVMSTGPIRNGDWTFQTVVMLEMTPELGHVYTCLVDHSSLLSPVSVEWRAQSEYSWRKMLSGIAAFLLGLIFLLVGIVIQLRAQKGYVRTQMSGNEVSRAVLLPQSC

SEQ ID NO: 56 - DNA, 4507 bp, Artificial Sequence
  Synthetic
ctgcgcgctcgctcgctcactgaggccgcccgggcaaagcccgggcgtcgggcgacctttggtcgcccggcctcagtgagcgagcgagcgcgcagagagggagtggccaactccatcactaggggttcctgcggccgcggtcgagtatcaagttgctttctgtcccggcagaggaagccagatcgctgagggtccggtctccagtttgcctcctgctatatccattggaagagaaaagtttgtgacttgggcccccaagttttgagagaactgggctttcggcgcggggggacagaggaggctcgtggggaggtgagtggacctcctggatcgatttaggaggctcgggtgggactgggaccaatcgcacctttgttgagccgtcactcattatggggagcccctcccaacaaccatagcgaatatttattgagctccacgcttagcagatcccccgataagctatgtacagacataattcgttgtaggtctcatttccacattttgtcgtggaggaaactgaggctcaaaggttaagtcacgtgcccaagttctcacggcctataaattgagggattcgaacccagacagctgaccccagagccccggcttttttttcctttcttttttttttttttttttttttttgagacagagtcttgctctgtcgccccagctacagtgcagtggtgcgatctctgctcaccgcaacctccacctcccgagttcaagcaattctgcctcagcctcccgagtagctgggatcacaggcgcccgccaccgcgcttggctaatttttgtatttttagtacagatggggtttcaccatggtggccagcctggtctcgaactcctgacctcatgatccaccctcctcggcctcccaaagtgctgggattacagccgtgagccactgtgccctgccagagcccaggctcttaaacattgcacattgtaggtgctttggtggtggggaatggtagacctcgaaagcagttggactctggttttcatttccctggctctggtaattaacctggacctcagtttacccaccctcacagtgcaaggctaggtatgcagtcggtgcctactttattataactgttgataattattgtcatctctccccttctgacacctccgccagctttccccatctagataacttcgtataatgtatgctatacgaagttatggatccatcgattctgcgatcgctccggtgcccgtcagtgggcagagcgcacatcgcccacagtccccgagaagttggggggaggggtcggcaattgaaccggtgcctagagaaggtggcgcggggtaaactgggaaagtgatgtcgtgtactggctccgcctttttcccgagggtgggggagaaccgtatataagtgcagtagtcgccgtgaacgttctttttcgcaacgggtttgccgccagaacacagctgaagcttccaccatgcccacgctactgcgggtttatatagacggtccccacgggatggggaaaaccaccaccacgcaactgctggtggccctgggttcgcgcgacgatatcgtctacgtacccgagccgatgacttactggcgggtgctgggggcttccgagacaatcgcgaacatctacaccacacaacaccgcctcgaccagggtgagatatcggccggggacgcggcggtggtaatgacaagcgcccagataacaatgggcatgccttatgccgtgaccgacgccgttctggctcctcatatcgggggggaggctgggagctcacatgccccgcccccggccctcaccctcatcttcgaccgccatcccatcgccgccctcctgtgctacccggccgcgcggtaccttatgggcagcatgaccccccaggccgtgctggcgttcgtggccctcatcccgccgaccttgcccggcaccaacatcgtgcttggggcccttccggaggacagacacatcgaccgcctggccaaacgccagcgccccggcgagcggctggacctggctatgctggctgcgattcgccgcgtttacgggctacttgccaatacggtgcggtatctgcagtgcggcgggtcgtggcgggaggactggggacagctttcggggacggccgtgccgccccagggtgccgagccccagagcaacgcgggcccacgaccccatatcggggacacgttatttaccctgtttcgggcccccgagttgctggcccccaacggcgacctgtataacgtgtttgcctgggccttggacgtcttggccaaacgcctccgttccatgcacgtctttatcctggattacgaccaatcgcccgccggctgccgggacgccctgctgcaacttacctccgggatggtccagacccacgtcaccacccccggctccataccgacgatatgcgacctggcgcgcacgtttgcccgggagatgggatcggccattgaacaagatggattgcacgcaggttctccggccgcttgggtggagaggctattcggctatgactgggcacaacagacaatcggctgctctgatgccgccgtgttccggctgtcagcgcaggggcgcccggttctttttgtcaagaccgacctgtccggtgccctgaatgaactgcaggacgaggcagcgcggctatcgtggctggccacgacgggcgttccttgcgcagctgtgctcgacgttgtcactgaagcgggaagggactggctgctattgggcgaagtgccggggcaggatctcctgtcatctcaccttgctcctgccgagaaagtatccatcatggctgatgcaatgcggcggctgcatacgcttgatccggctacctgcccattcgaccaccaagcgaaacatcgcatcgagcgagcacgtactcggatggaagccggtcttgtcgatcaggatgatctggacgaagagcatcaggggctcgcgccagccgaactgttcgccaggctcaaggcgcgcatgcccgacggcgaggatctcgtcgtgacccatggcgatgcctgcttgccgaatatcatggtggaaaatggccgcttttctggattcatcgactgtggccggctgggtgtggcggaccgctatcaggacatagcgttggctacccgtgatattgctgaagagcttggcggcgaatgggctgaccgcttcctcgtgctttacggtatcgccgctcccgattcgcagcgcatcgccttctatcgccttcttgacgagttcttctgagggtctctagcataacttcgtataatgtatgctatacgaagttataataaaagatccttattttcattggatctgtgtgttggttttttgtgtgggatccgttgactgagtcgacggagcttacccagcctgcagaagacctcatccagacccagcagacccctgcctcagaacttggggaccctgaagaccccggagaggaggctgcagatggctcagacactgtggtcctcagtctctttccctgcacccctgagcctgtgaatcctgaaccggatgccagtgtttcctctccacagggtaggatacctcctctgggattagccctctgggattccatgatgatggaatgtcaggcctcacatggaacctgtgtcttgctttcgtttttgttttgttttgttttgttgttttttgagatggagttttgctcttgttgcccatgctggagtgcaatggcgtgatctcagctcactgcaacctctgcctcctgggttcaactgattctcctgtctcagcctcctgagtagctgggattacaggcttccgccactacgcccagctaattttttgggtatttttagtagagacggggtttcaccatgttggccaggctggtcttgaactcctgacctcaggtgatccgcccacctcggcctcccaaagtgctgggattacaggcatgagccactgtgcccggcctgtttttgttttttgatacagggtctcgctctgttactaaggctggagtgcagtgatgcaatcatagttcactgcagcctcaacttcctgggctgaagccatcactcagcctccctaggagctgggactataggcatgcaaccacacctggctaattttttttttttttttgggaggctggtctccacctcctgggctcaagtgatctgcaggcctccacttccgaaagtgctgggattacaggtgtgagccacagtgcccggcccttcacacctgtttttaactctttgagggtagatagctaggagtgaaattactgggtcagatggtcatcctgttttacttactgaggaactgaggatttatttttgattggagtccaagaatatgcctaatttaggcggccgatcactagtgaattcgcggccgcaggaacccctagtgatggagttggccactccctctctgcgcgctcgctcgctcactgaggccgggcgaccaaaggtcgcccgacgcccgggctttgcccgggcggcctcagtgagcgagcgagcgcgcag